European Patent Specification EP 4 089 183 B1, published September 9, 2026. Title: HCBI, MSBI, MSSI and CMI sequences as an early marker for the future development of cancer and diseases of the CNS and as a target for the treatment and prevention of these diseases. Applicant: Deutsches Krebsforschungszentrum. The sequence listing filed with the application follows.

SEQUENCE LISTING (248 sequences)

SEQ ID NO: 1 - DNA, 2544 bp, Artificial Sequence
  source 1..2544: /mol_type="DNA" /note="HCBI6.252" /organism="Artificial Sequence"
ttttgtttttcaaaggaagtaattagcgagtgtctacgagcgacacaatgaaagttcgattattccctcctctaaaaaaccgcttttaaaaatattggttgctagatggttttaactatcgtgagcttttgcttttaaaaatacacgagcaaagcgagttcatagtcgcttttgatctgctcttactaacagctcatttttaatgggccgttagtaagagatgcttttggggtttcggggcttgccctgaacaaggtcacaaagtgggaatttatcacggtagtgaaaaagtaccctttgtgtatccttgctttatgctttttaaacctttgaacttttcccttaatttgcagaaattgcccctcgactaagcttgcttagtcaaaaaagtttgagcaaagcgaaaacatagggcaattttcatgatgaaaatgggcttttaaagtttttaaatgcttttaaatgcttttagacatgttgaaatgcaagcctagcaaggcatacagaggacatacccctacgtttaccgatcaatacccctacgtttaccgatcaatacccctacgtttaccgatcaatacccctacgtttaccttgcatatcactacaaacaatattaatgtagtaataacttcaaaataataaatgtaggttatgagcgatttaatagtaaaagataacgccctaatgaacgctagttacaacttagctttggttgaacagcgtttaatccttttagctatattggaagcgagagaaacaggcaaagggattaatgccaatgatcccttaacagttcatgcaagtagctatatcaatcaatttaacgtggaaagacatacggcatatcaagcattaaaagatgcttgcaaagacttgtttgcacgtcaatttagttaccaagaaaagcgagaacgtggacgaattaatattacaagtcgatgggtttcacaaattggttatatggacgatacagcaaccgttgaaattatttttgcccctgcggttgttcctttgattacacgtttagaggaacaattcactcaatacgatattgaacaaattagcgagttatcgagtgcttatgctgtccgcctatatgagttactaatttgttggcgtagcacaggaaaaaccccaattattgatctaacagagtttagaaagcgtctaggtgttttagataccgaatacactagaacagataacttgaagatgcgagtgattgagctaggacttaaacaaatcaacgagcatacggacattacagcaagctacgaacagcacaaaaaagggcggacaatcacaggattctcattcaagtttaagcagaagaagaaaacaggggcggaaatgccaaaaaatagcgattctagcccacatatcgaaaaacctagtcaaatccctgccaacatcgcaaaacagcctgaaaatgccaaaaaagatgatttagggcacagagcaagcaagattacagggttaattatgtctgaatggtttagcagatcggtttaaacgtggtgatgagtcagtaatagacatgatgaaacgcatcaaagaggaaattacaactgatacaacagcagaccaatgggaaaacaagctagaagaatttggcgtgatttttcagtcatgatcaatttcccgaaggacatataaaaaataatgtagttaaatatagtagttataatattgactacaatatttaactactatattgtagtcttaaatcaacttacatagaatttaaattatgtctcttcgccaaattttagaacaatctctctttgatcaaactgatgaaagctctactgtgccactatcaattagacttccaaacaacttgaataatgagcttgaagaactgactataacactagataaatccaagagttttctactcctagagttcattaaggctggaattagtgagactagcaatatgttagaagacaaagcgaagaaccctatacttgaaagtccaagagattctagtgactttacaactcataagaagtttatgttgaacactaatttcaataacaataaagcatcacacatgactatgttggagaatcaagaagctgctgcatttcgtaaaggttggaaagaatatatctgtaatttagaagaaggcgataaggtttacctttatcaaagtggcgttggttttgtagcatctggtattgtcactggtgacttaatcaaaagtgagtatcgtggacaaccagaagaaaaatattctaaaaaataaaggattttaaaataggatttaaagcaatttctgcaaaagagtttaagaccttaactggcggtggtgctagctttcgtacaacaatgagcgagctaaagcctgaacaatgtagaaaattagatatggaaatagaaaaacggatgaagtcagtaagttaaaaatatgagttgttgttttagtgtgtcacgtagcaatcacttagaagttccctttgtattacttgtctagcaatggttttaaaaagcgtcactactgatagtgacgctttatacccctacgtttaccgatca

SEQ ID NO: 2 - DNA, 1331 bp, Artificial Sequence
  source 1..1331: /mol_type="DNA" /note="Sphinx 1.76" /organism="Artificial Sequence"
ttttaaacctttgaacttttcccttaatttgcagaaattgcccctcgactaagcttgcttagtcaaaaaagtttgagcaaagcgaaaacatagggcaattttcatgatgaaaatgggcttttaaagtttttaaatgcttttaaatgcttttagacatgttgaaatgcaagcctagcaaggcatacagaggacatacccctacgtttaccgatcaatacccctacgtttaccgatcaatacccctacgtttaccgatcaatacccctacgtttaccttgcatatcactacaaacaatattaatgtagtaataacttcaaaataataaatgtaggttatgagcgatttaatagtaaaagataacgccctaatgaacgctagttacaacttagctttggttgaacagcgtttaatccttttagctatattggaagcgagagaaacaggcaaagggattaatgccaatgatcccttaacagttcatgcaagtagctatatcaatcaatttaacgtggaaagacatacggcatatcaagcattaaaagatgcttgcaaagacttgtttgcacgtcaatttagttaccaagaaaagcgagaacgtggacgaattaatattacaagtcgatgggtttcacaaattggttatatggacgatacagcaaccgttgaaattatttttgcccctgcggttgttcctttgattacacgtttagaggaacaattcactcaatacgatattgaacaaattagcgagttatcgagtgcttatgctgtccgcctatatgagttactaatttgttggcgtagcacaggaaaaaccccaattattgatctaacagagtttagaaagcgtctaggtgttttagataccgaatacactagaacagataacttgaagatgcgagtgattgagctaggacttaaacaaatcaacgagcatacggacattacagcaagctacgaacagcacaaaaaagggcggacaatcacaggattctcattcaagtttaagcagaagaagaaaacaggggcggaaatgccaaaaaatagcgattctagcccacatatcgaaaaacctagtcaaatccctgccaacatcgcaaaacagcctgaaaatgccaaaaaagatgatttagggcacagagcaagcaagattacagggttaattatgtcgaatggtttagcagatcggtttaaacgtggtgatgagtcagtaatagacatgatgaaacgcatcaaagaggaaattacaactgatacaacagcagaccaatgggaaaacaagctagaagaatttggcgtgatttttcagtcatgatcaatttcccgaagg

SEQ ID NO: 3 - DNA, 1324 bp, Artificial Sequence
  source 1..1324: /mol_type="DNA" /note="subject" /organism="Artificial Sequence"
ttctaaacctttgacttcttccccattgtttgcagaaattgcccctcgaagcttgcttagtcaaaaaagtttgagcaaagcgaaaacatagggcaattttcatgaagaaattgggcttttaaagtttttaaatgttttaaatgcttttagacatgctaagaagcccacacagcaaggcatacagaggacattctcctacgtttaccgatcaatacccccgtttaccgatcaatacccctacgtttaccgatcaatacccctacgtttaccttgcgtataactacaaagaatactagtgtagtataacttcaaaagaataattgtaggttatgagcgatttaatagtaaaagataacgccctaatgaatgctagttataacttagctttggttgaacagaggttaattctattagcaatcatagaagcgagagaaacaggcaaagggattaatgccaatgatcctcttacggttcatgcaggtagctatatcaatcaatttaacgtacaaaggcatacggcatatcaagccctcaaagatgcttgtaaagacttgtttgcccgtcaattcagttaccaagaaaagcgagaacgaggacgaattaatattacaagtcgatgggtttcgcaaattggctatatggacgatacagcaaccgttgagattatttttgcccctgcggttgttcctctgattacacggctagaggaacagttcacccagtacgatattgagcaaattagcggtttatcgagtgcatatgctgttcgtatgtacgaactgctgatttgttggcgtagcacaggcaaaacaccaattattgagctagacgagtttagaaagcgaataggtgttttagatactgaatacactagaacagataatttaaagatgcaagttattgaattagccctaaaacaaatcaacgaacatactgacatcacagcaagctatgaacaacacaaaaaagggcgagtgattaccggattctcattcatgtttaagcacaagaaacaaaacagcgataaaacgcctgatactaacgcttctagcccacgtatcgtaaaacatagtcaaatccctaccaacattgtaaaacagcctgaaaacgccaaaatgagcgatttagaacatagagcgagccgtgttacaggggaaataatgcgaaatcgtctgtcagatcggtttaaacaaggcgatgaatcagcaatcgacatgatgaaacgtattcaaagtgaaataataaccgatgcaatagcagaccagtgggaaagcaaactggaggagtttggcgtggttttttagtcatgacgatttcccgaagg

SEQ ID NO: 4 - DNA, 153 bp, Artificial Sequence
  source 1..153: /mol_type="DNA" /note="query" /organism="Artificial Sequence"
attagcgagtgtctacgagcgacacaatgaaagttcgattattccctcctctaaaaaaccgcttttaaaaatattggttgctagatggttttaactatcgtgagcttttgcttttaaaaatacacgagcaaagcgagttcatagtcgcttttg

SEQ ID NO: 5 - DNA, 152 bp, Artificial Sequence
  source 1..152: /mol_type="DNA" /note="subject" /organism="Artificial Sequence"
attagcgagtgtctacgagcgactcaatgaaagttcgattattccccctctggaaaaccgcttttaaaaatattggctgctagatggtttttactatagtgaggttttgcttttaaaaaaacacgagcaaagcgagttcatagttgcttttg

SEQ ID NO: 6 - protein, 324 aa, Artificial Sequence
  SOURCE 1..324: /mol_type="protein" /note="query" /organism="Artificial Sequence"
MSDLIVKDNALMNASYNLALVEQRLILLAILEARETGKGINANDPLTVHASSYINQFNVERHTAYQALKDACKDLFARQFSYQEKRERGRINITSRWVSQIGYMDDTATVEIIFAPAVVPLITRLEEQFTQYDIEQISELSSAYAVRLYELLICWRSTGKTPIIDLTEFRKRLGVLDTEYTRTDNLKMRVIELGLKQINEHTDITASYEQHKKGRTITGFSFKFKQKKKTGAEMPKNSDSSPHIEKPSQIPANIAKQPENAKKDDLGHRASKITGLIMSNGLADRFKRGDESVIDMMKRIKEEITTDTTADQWENKLEEFGVIF

SEQ ID NO: 7 - protein, 324 aa, Artificial Sequence
  SOURCE 1..324: /mol_type="protein" /note="subject" /organism="Artificial Sequence"
MSDLIVKDNALMNASYNLALVEQRLILLAIIEARETGKGINANDPLTVHAGSYINQFNVQRHTAYQALKDACKDLFARQFSYQEKRERGRINITSRWVSQIGYMDDTATVEIIFAPAVVPLITRLEEQFTQYDIEQISGLSSAYAVRMYELLICWRSTGKTPIIELDEFRKRIGVLDTEYTRTDNLKMQVIELALKQINEHTDITASYEQHKKGRVITGFSFMFKHKKQNSDKTPDTNASSPRIVKHSQIPTNIVKQPENAKMSDLEHRASRVTGEIMRNRLSDRFKQGDESAIDMMKRIQSEIITDAIADQWESKLEEFGVVF

SEQ ID NO: 8 - protein, 324 aa, Artificial Sequence; identical to SEQ ID NO: 6
  SOURCE 1..324: /mol_type="protein" /note="query" /organism="Artificial Sequence"

SEQ ID NO: 9 - protein, 324 aa, Artificial Sequence
  SOURCE 1..324: /mol_type="protein" /note="subject" /organism="Artificial Sequence"
MSELIVKDNALMNASYNLDLVEQRLILLAIVEARESGKGINANDPLTVHAESYINQFGVHRTTAYQALKDACKDLFARQFSYQEKRERGRANITSRWVSQIAYIDETATVEIIFAPAVVPLITRLEKQFTQYDIEQISGLSSAYAVRMYELLICWRSTGKTPVIELGEFRKRIGVLDTEYIRTDNLKMRVIELALKQINDHTDITATYEQHKKGRTITGFSFKFKQKRKTELETPKNSDSDVPKQKSVEIPTNLVKQPENANMSDLQHRASKITGLIMSNRLSDRFKQSDESIMQMMARIQSEITDEAIANQWENKLEEFGVIF

SEQ ID NO: 10 - protein, 324 aa, Artificial Sequence; identical to SEQ ID NO: 7
  SOURCE 1..324: /mol_type="protein" /note="SPTREMBL:E5LG72 9ZZZZ" /organism="Artificial Sequence"

SEQ ID NO: 11 - DNA, 1613 bp, Artificial Sequence
  source 1..1613: /mol_type="DNA" /note="HCBI6.159" /organism="Artificial Sequence"
ttttgtttttcaaaggaagtaattggcgagtgtctacgagcgacacaatgaaagttcgattattccctcctctaaaaaaccgcttttaaaaatattggttgctagatggttttaactatcgtgagcttttgcttttaaaaatacacgagcaaagcgagttcatagtcgcttttgatctgctcttactaacagctcatttttaatgggccgttagtaagagatgcttttggggtttcggggcttgccctgaacaaggtcacaaagtgggaatttatcacggtagtgaaaaagtaccctttgtgtatccttgctttatgctttttaaacctttgaacttttcccttaatttgcagaaattgcccctcgactaagcttgcttagtcaaaaaagtttgagcaaagcgaaaacatagggcaattttcatgatgaaaatgggcttttaaagtttttaaatgcttttaaatgcttttagacatgttgaaatgcaagcctagcaaggcacacagaggacatacccctgcgtttaccgatcaatacccctacgtttaccgatcaatacccctacgtttaccgatcaatacccctacgtttaccttgcatatcactacaaacaatattaatgtagtaataacttcaaaataataaatgtaggttatgagcgatttaatagtaaaagataacgccctaatgaacgctagttacaacttagctttggttgaacagcgtttaatccttttagctatattggaagcgagagaaacaggcaaagggattaatgccaatgatcccttaacagttcatgcaagtagctatatcaatcaatttaacgtggaaagacatacggcatatcaagcattaaaagatgcttgcaaagacttgtttgcacgtcaatttagttaccaagaaaagcgagaacgtggacgaattaatattacaagtcgatgggtttcacaaattggttatatggacgatacagcaaccgttgaaattatttttgcccctgcggttgttcctttgattacacgtttagaggaacaattcactcaatacgatattgaacaaattagcgagttatcgagtgcttatgctgtccgcctatatgagttactaatttgttggcgtagcacaggactatgttggagaatcaagaagctgctgcatttcgtaaaggttggaaagaatatatctgtaatttagaagaaggcgataaggtttacctttatcaaagtggcgttggttttgtagcatctggtattgtcactggtgacttaatcaaaagtgagtatcgtggacaaccagaagaaaaatattctaaaaaattaaaggattttaaaataggatttaaagcaatttctgcaaaagagtttaagaccttaactggcggtggtgctagctttcgtacaacaatgagcgagctaaagcctgaacaatgtagaaaattagatatggaaatagaaaaacggatgaagtcagtaagttaaaaatatgagttgttgttttagtgtgtcacgtagcaatcacttagaagttccctttgtattacttgtctagcaatggttttaaaaagcgtcactactgatagtgacgctttatacccctacgtttaccgatca

SEQ ID NO: 12 - DNA, 811 bp, Artificial Sequence
  source 1..811: /mol_type="DNA" /note="query" /organism="Artificial Sequence"
ttttaaacctttgaacttttcccttaatttgcagaaattgcccctcgactaagcttgcttagtcaaaaaagtttgagcaaagcgaaaacatagggcaattttcatgatgaaaatgggcttttaaagtttttaaatgcttttaaatgcttttagacatgttgaaatgcaagcctagcaaggcacacagaggacatacccctgcgtttaccgatcaatacccctacgtttaccgatcaatacccctacgtttaccgatcaatacccctacgtttaccttgcatatcactacaaacaatattaatgtagtaataacttcaaaataataaatgtaggttatgagcgatttaatagtaaaagataacgccctaatgaacgctagttacaacttagctttggttgaacagcgtttaatccttttagctatattggaagcgagagaaacaggcaaagggattaatgccaatgatcccttaacagttcatgcaagtagctatatcaatcaatttaacgtggaaagacatacggcatatcaagcattaaaagatgcttgcaaagacttgtttgcacgtcaatttagttaccaagaaaagcgagaacgtggacgaattaatattacaagtcgatgggtttcacaaattggttatatggacgatacagcaaccgttgaaattatttttgcccctgcggttgttcctttgattacacgtttagaggaacaattcactcaatacgatattgaacaaattagcgagttatcgagtgcttatgctgtccgcctatatgagttactaatttgttggcgtagcacagg

SEQ ID NO: 13 - DNA, 805 bp, Artificial Sequence
  source 1..805: /mol_type="DNA" /note="subject" /organism="Artificial Sequence"
ttctaaacctttgacttcttccccattgtttgcagaaattgcccctcgaagcttgcttagtcaaaaaagtttgagcaaagcgaaaacatagggcaattttcatgaagaaattgggcttttaaagtttttaaatgttttaaatgcttttagacatgctaagaagcccacacagcaaggcatacagaggacattctcctacgtttaccgatcaatacccccgtttaccgatcaatacccctacgtttaccgatcaatacccctacgtttaccttgcgtataactacaaagaatactagtgtagtataacttcaaaagaataattgtaggttatgagcgatttaatagtaaaagataacgccctaatgaatgctagttataacttagctttggttgaacagaggttaattctattagcaatcatagaagcgagagaaacaggcaaagggattaatgccaatgatcctcttacggttcatgcaggtagctatatcaatcaatttaacgtacaaaggcatacggcatatcaagccctcaaagatgcttgtaaagacttgtttgcccgtcaattcagttaccaagaaaagcgagaacgaggacgaattaatattacaagtcgatgggtttcgcaaattggctatatggacgatacagcaaccgttgagattatttttgcccctgcggttgttcctctgattacacggctagaggaacagttcacccagtacgatattgagcaaattagcggtttatcgagtgcatatgctgttcgtatgtacgaactgctgatttgttggcgtagcacagg

SEQ ID NO: 14 - DNA, 153 bp, Artificial Sequence
  source 1..153: /mol_type="DNA" /note="query" /organism="Artificial Sequence"
attggcgagtgtctacgagcgacacaatgaaagttcgattattccctcctctaaaaaaccgcttttaaaaatattggttgctagatggttttaactatcgtgagcttttgcttttaaaaatacacgagcaaagcgagttcatagtcgcttttg

SEQ ID NO: 15 - DNA, 152 bp, Artificial Sequence; identical to SEQ ID NO: 5
  source 1..152: /mol_type="DNA" /note="subject" /organism="Artificial Sequence"

SEQ ID NO: 16 - DNA, 59 bp, Artificial Sequence
  source 1..59: /mol_type="DNA" /note="query" /organism="Artificial Sequence"
ctttttaaacctttgaacttttcccttaatttgcagaaattgcccctcgactaagcttg

SEQ ID NO: 17 - DNA, 59 bp, Artificial Sequence
  source 1..59: /mol_type="DNA" /note="subject" /organism="Artificial Sequence"
ctttttaaacctttcgactttccctatcctttgcataaattgcccctgacgtagcaaag

SEQ ID NO: 18 - protein, 159 aa, Artificial Sequence
  SOURCE 1..159: /mol_type="protein" /note="query" /organism="Artificial Sequence"
MSDLIVKDNALMNASYNLALVEQRLILLAILEARETGKGINANDPLTVHASSYINQFNVERHTAYQALKDACKDLFARQFSYQEKRERGRINITSRWVSQIGYMDDTATVEIIFAPAVVPLITRLEEQFTQYDIEQISELSSAYAVRLYELLICWRSTG

SEQ ID NO: 19 - protein, 159 aa, Artificial Sequence
  SOURCE 1..159: /mol_type="protein" /note="subject" /organism="Artificial Sequence"
MSDLIVKDNALMNASYNLALVEQRLILLAIIEARETGKGINANDPLTVHAGSYINQFNVQRHTAYQALKDACKDLFARQFSYQEKRERGRINITSRWVSQIGYMDDTATVEIIFAPAVVPLITRLEEQFTQYDIEQISGLSSAYAVRMYELLICWRSTG

SEQ ID NO: 20 - protein, 159 aa, Artificial Sequence; identical to SEQ ID NO: 18
  SOURCE 1..159: /mol_type="protein" /note="query" /organism="Artificial Sequence"

SEQ ID NO: 21 - protein, 159 aa, Artificial Sequence
  SOURCE 1..159: /mol_type="protein" /note="subject" /organism="Artificial Sequence"
MSELIVKDNALMNASYNLDLVEQRLILLAIVEARESGKGINANDPLTVHAESYINQFGVHRTTAYQALKDACKDLFARQFSYQEKRERGRANITSRWVSQIAYIDETATVEIIFAPAVVPLITRLEKQFTQYDIEQISGLSSAYAVRMYELLICWRSTG

SEQ ID NO: 22 - protein, 159 aa, Artificial Sequence; identical to SEQ ID NO: 18
  SOURCE 1..159: /mol_type="protein" /note="query" /organism="Artificial Sequence"

SEQ ID NO: 23 - protein, 160 aa, Artificial Sequence
  SOURCE 1..160: /mol_type="protein" /note="subject" /organism="Artificial Sequence"
MSELIVKDNALMNASYNLALVEQRLILLAIIEARESGRGINANDPLTVHAESYINQFKVEKHTAYQALKDACKDLFARQFSYQQRSAKGNTTNMTSRWISQIGYTENEATVQLVFAPAVVPLITRLEEQFTKYDIEQISSLSSAYAVRLYELLICWRSTG

SEQ ID NO: 24 - DNA, 1766 bp, Artificial Sequence
  source 1..1766: /mol_type="DNA" /note="MSBI1.176" /organism="Artificial Sequence"
aagcttgcttagtcaaaaaagtttgagcaaagcgaaaacatagggcaattttcatgaagaaattgggcttttaaagtttttaaatgcttttaaatgcttttagacatgctaagaagcccacacagcaaggcatacagaggacattctcctacgtttaccgatcaatacccctacgtttaccgatcaatacccctacgtttaccgatcaatacccctacgtttaccttgcgtataactacaaagaatactagtgtagtaataacttcaaaagaataattgtaggttatgagcgatttaatagtaaaagataacgccctaatgaatgctagttataacttagctttggttgaacagaggttaattctattagcaatcatagaagcgagagaaacaggcaaagggattaatgccaatgatcctttaacagttcatgcaagtagctatatcaatcaatttaacgtagaaaggcatacggcatatcaagccctcaaagatgcttgtaaagacttgtttgcccgtcaattcagttaccaagaaaagcgagaacgaggacgaattaatattacaagtcgatgggtttcgcaaattggctatatggacgatacagcaaccgttgagattatttttgcccctgcggttgttcctctgattacacggctagaggaacagttcacccagtacgatattgagcaaattagcggtttatcgagtgcatatgctgttcgtatgtacgaactgctgatttgttggcgtagcacaggcaaaacaccaattattgagctagacgagtttagaaagcgaataggtgttttagatactgaatacactagaacagataatttaaagatgcgagttattgaattagccctaaaacaaatcaacgaacatacagacatcacagcaagctatgaacaacacaaaaaagggcgagtgattacaggattctcattcaagtttaagcacaagaaacaaaacagcgataaaacgccaaaaaatagcgattctagcccacgtatcgtaaaacatagtcaaatccctaccaacattgtaaaacagcctgaaaacgccaaaatgagcgatttagaacatagagcgagccgtgttacaggggaaataatgcgaaatcgtctgtcagatcggtttaaacaaggcgatgaatcagcaatcgacatgatgaaacgtattcaaagtgaaataataaccgatgcaatagcagaccagtgggaaagcaaactggaggagtttggcgtggttttttagtcatgacgatttcccgaagggcgcacttagccattgagaaaaatcttcgattttttcaatggaagtccgtgggggtaaacccctcaaccccaaaagcaaaaacactgtaatcagggaaaaaacatttttgattttgatccttgtttgtcactcgtagacactcgttttgttttgctctttctagaattcacaaaaaagatattagcgagtgtctacgagcgactcaatgaaagttcgattattccccctctggaaaaccgcttttaaaaatattggctgctagatggtttttactatagtgaggttttgcttttaaaaaaacacgagcaaagcgagttcatagttgcttttgcttgttttcgggtcttaggggaaatcccctaacaagtcctcgaatatcaaaatgtggctacattttgtatatacgggtaggcttgcttatttgattttttttcttctaaacctttgacttcttccccattgtttgcagaaattgcccctcgact

SEQ ID NO: 25 - DNA, 1439 bp, Artificial Sequence
  source 1..1439: /mol_type="DNA" /note="query" /organism="Artificial Sequence"
aagcttgcttagtcaaaaaagtttgagcaaagcgaaaacatagggcaattttcatgaagaaattgggcttttaaagtttttaaatgcttttaaatgcttttagacatgctaagaagcccacacagcaaggcatacagaggacattctcctacgtttaccgatcaatacccctacgtttaccgatcaatacccctacgtttaccgatcaatacccctacgtttaccttgcgtataactacaaagaatactagtgtagtaataacttcaaaagaataattgtaggttatgagcgatttaatagtaaaagataacgccctaatgaatgctagttataacttagctttggttgaacagaggttaattctattagcaatcatagaagcgagagaaacaggcaaagggattaatgccaatgatcctttaacagttcatgcaagtagctatatcaatcaatttaacgtagaaaggcatacggcatatcaagccctcaaagatgcttgtaaagacttgtttgcccgtcaattcagttaccaagaaaagcgagaacgaggacgaattaatattacaagtcgatgggtttcgcaaattggctatatggacgatacagcaaccgttgagattatttttgcccctgcggttgttcctctgattacacggctagaggaacagttcacccagtacgatattgagcaaattagcggtttatcgagtgcatatgctgttcgtatgtacgaactgctgatttgttggcgtagcacaggcaaaacaccaattattgagctagacgagtttagaaagcgaataggtgttttagatactgaatacactagaacagataatttaaagatgcgagttattgaattagccctaaaacaaatcaacgaacatacagacatcacagcaagctatgaacaacacaaaaaagggcgagtgattacaggattctcattcaagtttaagcacaagaaacaaaacagcgataaaacgccaaaaaatagcgattctagcccacgtatcgtaaaacatagtcaaatccctaccaacattgtaaaacagcctgaaaacgccaaaatgagcgatttagaacatagagcgagccgtgttacaggggaaataatgcgaaatcgtctgtcagatcggtttaaacaaggcgatgaatcagcaatcgacatgatgaaacgtattcaaagtgaaataataaccgatgcaatagcagaccagtgggaaagcaaactggaggagtttggcgtggttttttagtcatgacgatttcccgaagggcgcacttagccattgagaaaaatcttcgattttttcaatggaagtccgtgggggtaaacccctcaaccccaaaagcaaaaacactgtaatcagggaaaaaacatttttgattttgatccttgtttgtcactcgtagacactcgttttgttttgctctt

SEQ ID NO: 26 - DNA, 1434 bp, Artificial Sequence
  source 1..1434: /mol_type="DNA" /note="subject" /organism="Artificial Sequence"
aagcttgcttagtcaaaaaagtttgagcaaagcgaaaacatagggcaattttcatgaagaaattgggcttttaaagtttttaaatgttttaaatgcttttagacatgctaagaagcccacacagcaaggcatacagaggacattctcctacgtttaccgatcaatacccccgtttaccgatcaatacccctacgtttaccgatcaatacccctacgtttaccttgcgtataactacaaagaatactagtgtagtataacttcaaaagaataattgtaggttatgagcgatttaatagtaaaagataacgccctaatgaatgctagttataacttagctttggttgaacagaggttaattctattagcaatcatagaagcgagagaaacaggcaaagggattaatgccaatgatcctcttacggttcatgcaggtagctatatcaatcaatttaacgtacaaaggcatacggcatatcaagccctcaaagatgcttgtaaagacttgtttgcccgtcaattcagttaccaagaaaagcgagaacgaggacgaattaatattacaagtcgatgggtttcgcaaattggctatatggacgatacagcaaccgttgagattatttttgcccctgcggttgttcctctgattacacggctagaggaacagttcacccagtacgatattgagcaaattagcggtttatcgagtgcatatgctgttcgtatgtacgaactgctgatttgttggcgtagcacaggcaaaacaccaattattgagctagacgagtttagaaagcgaataggtgttttagatactgaatacactagaacagataatttaaagatgcaagttattgaattagccctaaaacaaatcaacgaacatactgacatcacagcaagctatgaacaacacaaaaaagggcgagtgattaccggattctcattcatgtttaagcacaagaaacaaaacagcgataaaacgcctgatactaacgcttctagcccacgtatcgtaaaacatagtcaaatccctaccaacattgtaaaacagcctgaaaacgccaaaatgagcgatttagaacatagagcgagccgtgttacaggggaaataatgcgaaatcgtctgtcagatcggtttaaacaaggcgatgaatcagcaatcgacatgatgaaacgtattcaaagtgaaataataaccgatgcaatagcagaccagtgggaaagcaaactggaggagtttggcgtggttttttagtcatgacgatttcccgaagggcgcacttagccattgagaaaaatcttcgattttttcaatggaagtccgtgggggtaaacccctcaaccccaaaagcaaaaacactgtaatcagggaaaaaacatttttgattttgatccttgtttgcactcgtagacactcgttttgttttgctctt

SEQ ID NO: 27 - DNA, 325 bp, Artificial Sequence
  source 1..325: /mol_type="DNA" /note="query" /organism="Artificial Sequence"
tctagaattcacaaaaaagatattagcgagtgtctacgagcgactcaatgaaagttcgattattccccctctggaaaaccgcttttaaaaatattggctgctagatggtttttactatagtgaggttttgcttttaaaaaaacacgagcaaagcgagttcatagttgcttttgcttgttttcgggtcttaggggaaatcccctaacaagtcctcgaatatcaaaatgtggctacattttgtatatacgggtaggcttgcttatttgattttttttcttctaaacctttgacttcttccccattgtttgcagaaattgcccctcga

SEQ ID NO: 28 - DNA, 325 bp, Artificial Sequence; identical to SEQ ID NO: 27
  source 1..325: /mol_type="DNA" /note="subject" /organism="Artificial Sequence"

SEQ ID NO: 29 - protein, 324 aa, Artificial Sequence
  SOURCE 1..324: /mol_type="protein" /note="query" /organism="Artificial Sequence"
MSDLIVKDNALMNASYNLALVEQRLILLAIIEARETGKGINANDPLTVHASSYINQFNVERHTAYQALKDACKDLFARQFSYQEKRERGRINITSRWVSQIGYMDDTATVEIIFAPAVVPLITRLEEQFTQYDIEQISGLSSAYAVRMYELLICWRSTGKTPIIELDEFRKRIGVLDTEYTRTDNLKMRVIELALKQINEHTDITASYEQHKKGRVITGFSFKFKHKKQNSDKTPKNSDSSPRIVKHSQIPTNIVKQPENAKMSDLEHRASRVTGEIMRNRLSDRFKQGDESAIDMMKRIQSEIITDAIADQWESKLEEFGVVF

SEQ ID NO: 30 - protein, 324 aa, Artificial Sequence; identical to SEQ ID NO: 7
  SOURCE 1..324: /mol_type="protein" /note="subject" /organism="Artificial Sequence"

SEQ ID NO: 31 - protein, 324 aa, Artificial Sequence; identical to SEQ ID NO: 29
  SOURCE 1..324: /mol_type="protein" /note="query" /organism="Artificial Sequence"

SEQ ID NO: 32 - protein, 324 aa, Artificial Sequence; identical to SEQ ID NO: 9
  SOURCE 1..324: /mol_type="protein" /note="subject" /organism="Artificial Sequence"

SEQ ID NO: 33 - DNA, 1766 bp, Artificial Sequence
  source 1..1766: /mol_type="DNA" /note="MSBI2.176" /organism="Artificial Sequence"
aagcttgcttagtcaaaaaagtttgagcaaagcgaaaacatagggcaattttcgtgatgaaaatgggcttttaatgtttttaaatgcttttaaatgcttttagacatgctgaaacgcttatatagcaatgcatacagaggacatatgtccacgtttacctatcaatatgtccacgtttacctatcaatatgtccacgtttacctatcaatatgtccacgtttaccttgcgtatttacacacatttaaatagtatggatatatccaatgaaattataatgtgtacttatgagcaaattagtagtgaaagacaatgccctaatgaacgctagttacaacttggatctcgttgaacagcgtttaattctattggcaatcatcgaagcaagagaatcaggcaaaggaattaatgcaaatgacccgcttacggttcatgcagagagttatatcaatcaatttggtgttcatcgagtaactgcatatcaagctctcaaagatgcttgtgataacttgtttgcacgtcaattcagctaccaatccaaaagtgaaaaagggaacatacaaaatcatcgttcacgttgggttagtgaaattatttacattgatacagaagcaacagtaaaaataatatttgcacctgctattgtcccactgattacaaggctagaagaacagttcaccaagtatgatattgagcaaattagtgatttatcgagtgcttatgcaattcgcttatacgagttattgatttgctggcgtagcacagggaaaacaccaattattgggctaggcgaatttagaaatcgggttggtgtgttagatagtgaatatcatcgaattgcacacttgaaagaacgagttattgaacattcaattaaacagattaacgagcataccgacatcacagccacctacgaacagcacaaaaaagggcggacaatcacaggattttcattcaagtttaagcagaagaagcccaaacaagccgaaattgctacagaaacgccaaaaacagccacgaatgacccagacacgacaaaaccccttacagagcctcagatcgcaaaatacagcatgattctgtgcaaactaggcagtatttcagacttgagtaacttcccagactatccagcttttgcaaattggattgggaacattttgaggaaccctgaaaaagcagatgaacaaatagcaaaacggattttcacagcattgaaaacagaaaccgactacagcaagaaaaactaatttttagttgtgatgggttttcccgaaataacatgaagggcgcacttacgcaaaatttttgctacgccaaattttgcaagtacggtcagggaaaccccgacaccccaaaagcaaaaacactgtaatcagggaaaaaacatttttgattttgatccttgtttgtcactcgtagacactcgttttgttttgctctttctagaattcacaaaaaagatattagcgagtgtctacgagcgactcaatgaaagttcgattattccccctctggaaaaccgcttttaaaaatattggctgctagatggtttttactatagtgaggttttgcttttaaaaaaacacgagcaaagcgagttcatagttgcttttgcttgttttcgggtcttaggggaaatcccctaacaagtcctcgaatatcaaaatgtggctacattttgtatatacgggtaggcttgcttatttgattttttttcttctaaacctttgacttcttccccattgtttgcagaaatgccccccgacc

SEQ ID NO: 34 - DNA, 1284 bp, Artificial Sequence
  source 1..1284: /mol_type="DNA" /note="query" /organism="Artificial Sequence"
agtcaaaaaagtttgagcaaagcgaaaacatagggcaattttcgtgatgaaaatgggcttttaatgtttttaaatgcttttaaatgcttttagacatgctgaaacgcttatatagcaatgcatacagaggacatatgtccacgtttacctatcaatatgtccacgtttacctatcaatatgtccacgtttacctatcaatatgtccacgtttaccttgcgtatttacacacatttaaatagtatggatatatccaatgaaattataatgtgtacttatgagcaaattagtagtgaaagacaatgccctaatgaacgctagttacaacttggatctcgttgaacagcgtttaattctattggcaatcatcgaagcaagagaatcaggcaaaggaattaatgcaaatgacccgcttacggttcatgcagagagttatatcaatcaatttggtgttcatcgagtaactgcatatcaagctctcaaagatgcttgtgataacttgtttgcacgtcaattcagctaccaatccaaaagtgaaaaagggaacatacaaaatcatcgttcacgttgggttagtgaaattatttacattgatacagaagcaacagtaaaaataatatttgcacctgctattgtcccactgattacaaggctagaagaacagttcaccaagtatgatattgagcaaattagtgatttatcgagtgcttatgcaattcgcttatacgagttattgatttgctggcgtagcacagggaaaacaccaattattgggctaggcgaatttagaaatcgggttggtgtgttagatagtgaatatcatcgaattgcacacttgaaagaacgagttattgaacattcaattaaacagattaacgagcataccgacatcacagccacctacgaacagcacaaaaaagggcggacaatcacaggattttcattcaagtttaagcagaagaagcccaaacaagccgaaattgctacagaaacgccaaaaacagccacgaatgacccagacacgacaaaaccccttacagagcctcagatcgcaaaatacagcatgattctgtgcaaactaggcagtatttcagacttgagtaacttcccagactatccagcttttgcaaattggattgggaacattttgaggaaccctgaaaaagcagatgaacaaatagcaaaacggattttcacagcattgaaaacagaaaccgactacagcaagaaaaactaatttttagttgtgatgggttttcccgaaataacatgaagggcgcactta

SEQ ID NO: 35 - DNA, 1283 bp, Artificial Sequence
  source 1..1283: /mol_type="DNA" /note="subject" /organism="Artificial Sequence"
agtcaaaaaagtttgagagaagcgaaaacatagggcaatttcatggtgagaatgggcttttaaggtttttaaaagcttttaaatgcttttagacatgctgaaacgaccacacagcaaggcatacagagggcatatgtccacgtttacctatcaatatgtccacgtttacctatcaatatgtccacgtttacctatcaatatgtccacgtttaccttgcatagtcacacatatttaaataatatggatatatccaataaaattataatgtgtacttatgagtaggttagtagtgaaagacaatgccctaatgaacgctagttataacttggatctcgttgaacagcgtttaatcctattggcaatcatcgaagcgagggagtcaggcaaaggaattaacgccaatgaccctctaacaatccatgcagagagctacatcaatcaatttggtgttcatcgagtaactgcatatcaagctctcaaagatgcttgtgataacctgtttgcacgtcaattcagctatcagtccaaaagtgaaaaaggaaacatacaaaatcatcgttcacgctgggttagtgaaattatttacatcgacacagaagcaacagtaaaaataatctttgcacctgctatcgtcccactgattacaagattagaagaacagttcaccaagtatgatattcagcaaattagtgatttatcgagtgcttatgcaatccgcttatacgaattattgatttgttggcgtagcacagggaaaacgccaattattgaattagctgaatttaggaatcgggttggtgtgttagatactgaatatcatcgaattgcccacttgaaagagcgagttattgaacattcaattaaacaaattaacgaacataccgacatcacagcgacctacgaacagcataaaaaagggcgagtgattacagggttctcattcaaatttaagcagaagaagcccaaacaagccgagattgccacagaaacgcccaaaacagccacgaatgacctagatacgataaaaccccttacagagccacagatcgcaaaatacagcatgattctgtgcaaactaggcagtatttcagacttgagtaacttcccagactatccagcttttgcaaattggattgggaacattttgaggaaccctgaaaaagcagatgaacaaatagcaaaacggattttcacagcattgaaaacagaaaccgactacagcaagaaaaactaatttttagttgtgatgggttttcccgaaataacatgaagggcgcactta

SEQ ID NO: 36 - DNA, 125 bp, Artificial Sequence
  source 1..125: /mol_type="DNA" /note="query" /organism="Artificial Sequence"
cctaacaagtcctcgaatatcaaaatgtggctacattttgtatatacgggtaggcttgcttatttgattttttttcttctaaacctttgacttcttccccattgtttgcagaaatgccccccgac

SEQ ID NO: 37 - DNA, 125 bp, Artificial Sequence
  source 1..125: /mol_type="DNA" /note="subject" /organism="Artificial Sequence"
cctaacaagtccccgaatatcaaaatgtggctacattttgtatatacgggtaggcttgcttattgaatctaattcctttttaaacctttcgactttccctatcctttgcataaattgcccctgac

SEQ ID NO: 38 - DNA, 885 bp, Artificial Sequence
  source 1..885: /mol_type="DNA" /note="query" /organism="Artificial Sequence"
attaacgagcataccgacatcacagccacctacgaacagcacaaaaaagggcggacaatcacaggattttcattcaagtttaagcagaagaagcccaaacaagccgaaattgctacagaaacgccaaaaacagccacgaatgacccagacacgacaaaaccccttacagagcctcagatcgcaaaatacagcatgattctgtgcaaactaggcagtatttcagacttgagtaacttcccagactatccagcttttgcaaattggattgggaacattttgaggaaccctgaaaaagcagatgaacaaatagcaaaacggattttcacagcattgaaaacagaaaccgactacagcaagaaaaactaatttttagttgtgatgggttttcccgaaataacatgaagggcgcacttacgcaaaatttttgctacgccaaattttgcaagtacggtcagggaaaccccgacaccccaaaagcaaaaacactgtaatcagggaaaaaacatttttgattttgatccttgtttgtcactcgtagacactcgttttgttttgctctttctagaattcacaaaaaagatattagcgagtgtctacgagcgactcaatgaaagttcgattattccccctctggaaaaccgcttttaaaaatattggctgctagatggtttttactatagtgaggttttgcttttaaaaaaacacgagcaaagcgagttcatagttgcttttgcttgttttcgggtcttaggggaaatcccctaacaagtcctcgaatatcaaaatgtggctacattttgtatatacgggtaggcttgcttatttgattttttttcttctaaacctttgacttcttccccattgtttgcagaaatgccccccgac

SEQ ID NO: 39 - DNA, 890 bp, Artificial Sequence
  source 1..890: /mol_type="DNA" /note="subject" /organism="Artificial Sequence"
atcaacgagcacaccgacatcacagccacctacgaacagcacaaaaaagggcggacaatcacaggattttcattcaagtttaagcagaagaagcccaaacaagccgaaattgctacagaaacgccaaaaacagccacgaatgacccagacacgacaaaaccccttacagagcctcagatcgcaaaatacagcatgattctgtgcaaactaggcagtatttcagacttgagtaacttcccagactatccagcttttgcaaattggattgggaacattttgaggaaccctgaaaaagcagatgaacaaatagcaaaacggattttcacagcattgaaaacagaaaccgactacagcaagaaaaactaatttttagttgtgatgggttttcccgaaataacatgaagggcgcacttagccattgagaaaaatcttcgattttttcaatggaagtccgtgggggtaaacccctcaaccccaaaagcaaaaacactgtaatcagggaaaaaacatttttgattttgatccttgtttgtcactcgtagacactcgttttgttttgctctttctagaattcacaaaaaagatattagcgagtgtctacgagcgactcaatgaaagttcgattattccccctctggaaaaccgcttttaaaaatattggctgctagatggtttttactatagtgaggttttgcttttaaaaaaacacgagcaaagcgagttcatagttgcttttgcttgttttcgggtcttaggggaaatcccctaacaagtcctcgaatatcaaaatgtggctacattttgtatatacgggtaggcttgcttatttgattttttttcttctaaacctttgacttcttccccattgtttgcagaaattgcccctcgac

SEQ ID NO: 40 - DNA, 324 bp, Artificial Sequence
  source 1..324: /mol_type="DNA" /note="query" /organism="Artificial Sequence"
aagcttgcttagtcaaaaaagtttgagcaaagcgaaaacatagggcaattttcgtgatgaaaatgggcttttaatgtttttaaatgcttttaaatgcttttagacatgctgaaacgcttatatagcaatgcatacagaggacatatgtccacgtttacctatcaatatgtccacgtttacctatcaatatgtccacgtttacctatcaatatgtccacgtttaccttgcgtatttacacacatttaaatagtatggatatatccaatgaaattataatgtgtacttatgagcaaattagtagtgaaagacaatgccctaatgaa

SEQ ID NO: 41 - DNA, 324 bp, Artificial Sequence
  source 1..324: /mol_type="DNA" /note="subject" /organism="Artificial Sequence"
aagcttgcttagtcaaaaaagtttgagcaaagcgaaaacatagggcaattttcgtgatgaaaatgggcttttaatgtttttaaatgcttttaaatgcttttagacatgctgaaacgcttatatagcaatgcatacagaggacatatgtccacgtttacctatcaatatgtccacgtttacctatcaatatgtccacgtttacctatcaatatgtccacgtttaccttgcgtatttacacacatttaaatagtatggatatatccaatgagattataatgtgtacttatgagcaaattagtagtgaaagacaatgccctaatcaa

SEQ ID NO: 42 - protein, 319 aa, Artificial Sequence
  SOURCE 1..319: /mol_type="protein" /note="query" /organism="Artificial Sequence"
MSKLVVKDNALMNASYNLDLVEQRLILLAIIEARESGKGINANDPLTVHAESYINQFGVHRVTAYQALKDACDNLFARQFSYQSKSEKGNIQNHRSRWVSEIIYIDTEATVKIIFAPAIVPLITRLEEQFTKYDIEQISDLSSAYAIRLYELLICWRSTGKTPIIGLGEFRNRVGVLDSEYHRIAHLKERVIEHSIKQINEHTDITATYEQHKKGRTITGFSFKFKQKKPKQAEIATETPKTATNDPDTTKPLTEPQIAKYSMILCKLGSISDLSNFPDYPAFANWIGNILRNPEKADEQIAKRIFTALKTETDYSKKN

SEQ ID NO: 43 - protein, 312 aa, Artificial Sequence
  SOURCE 1..312: /mol_type="protein" /note="subject" /organism="Artificial Sequence"
MRELVVKDNALINASYNLDLVEQRLILLAIVEARESGKGINANDPLVVHAESYINQFNVHRNTAYQALKDACHDLFVRQFSYQKVNDRGNVEHYRSRWVSEIGYVDNEAIVKLIFAPAIVPLITRLEEQFTKYELQQVSQLTSAYAVRLYELLIAWRSTGKTPVIELADFRKRIGILETEYKRMERFKTSVLELAINQINEHTDINVAYEQHKKGRSIVGFSFNFSQKEKKKILEKAQVSEGFKKLTEAQITKYSTVLSKLHELSDLSTFQDYQSFSIWIGNILREPESVRFETAERIFSSLFKRTDFASPN

SEQ ID NO: 44 - protein, 319 aa, Artificial Sequence; identical to SEQ ID NO: 42
  SOURCE 1..319: /mol_type="protein" /note="query" /organism="Artificial Sequence"

SEQ ID NO: 45 - protein, 312 aa, Artificial Sequence; identical to SEQ ID NO: 43
  SOURCE 1..312: /mol_type="protein" /note="subject" /organism="Artificial Sequence"

SEQ ID NO: 46 - DNA, 2521 bp, Artificial Sequence
  source 1..2521: /mol_type="DNA" /note="CMI1.252" /organism="Artificial Sequence"
ttaaaaatattggttgctagatggttttaactatcgtggagcttttgcttttaaaaatacacgaagcaaagcgagttcatagtcgcttttgatctgctcttactaacagctcatttttaatgggccgttagtaagagatgcttttggggtttcggggcttgccctgaacaaggtcacaaagtgggaatttatcacggtagtgaaaaagtaccctttgtgtatccttgctttatgctttttaaacctttggacttttcccttaatttgcagaaattgcccctcgactaagcaagcttagtcaaaaaagtttgagcaaagcgaaaacatagggcaattttcatgatgaaaatgggcttttaaagtttttaaatgcttttaaatgcttttagacatgttgaaatgcaagcctagcaaggcatacagaggacatacccctacgtttaccgatcaatacccctacgtttaccgatcaatacccctacgtttaccgatcaatacccctacgtttaccttgcatatcactacaaacaatattaatgtagtaataacttcaaaataataaatgtaggttatgagcgatttaatagtaaaggataacgccctaatgaacgctagttacaacttagctttggttgaacagcgtttaatccttttagctatattggaagcgagagaaacaggaaaagggattaatgccaatgaccccttaacagttcatgcaagtagctatatcaatcaatttaacgtggaaagacatacggcatatcaagcattaaaagatgcttgcaaagacttgtttgcacgtcaatttagttaccaagaaaagcgagaacgaggacgaattaatattacaagtcgatgggtttcacaaattggttatatggacgatacagcaaccgttgaaattatttttgcccctgcggttgttcctttgattacacgtttagaggaacaattcactcaatacgatattgaacaaattagcgagttatcgagtgcttatgctgtccgcctatatgagttactaatttgttggcgtagcacaggaaaaaccccaattattgatctaacagagtttagaaagcgtctaggcgttttagataccgaatacactaggacagataacttgaagatgcgagtgattgagctaggacttaaacaaatcaacgagcatacggacattacagcaagctacgaacagcacaaaaaagggcggacaatcacaggattctcattcaagtttaagcagaagaagaaaacaggggcggaaatgccaaaaaatagcgattctagcccacatatcgaaaaacctagtcaaatccctgccaacatcgcaaaacagcctgaaaatgccaaaaaagatgatttagggcacagagcaagcaagattacagggttaattatgtcgaatggtttagcagatcggtttaaacgtggtgatgagtcagtaatagacatgatgaaacgcatcgaggaaattacaactgatacaacagcagaccaatgggaaaacaagctagaagaatttggcgtgatttttcagtcatgatcaatttcccgaaggacatataaaaaataatgtagttaaatatagtagttataatattgactacaatatttaactactatattgtagtcttaaatcaacttacatagaatttaaattatgtctcttcgccaaattttagaacaatctctctttgatcaaactgatgaaagctctactgtgccactatcaattagacttccaaacaacttgaataatgagcttgaagaactgactataacactagataaatccaagagttttctactcctagagttcattaaggctggaattagtgagactagcaatatgttagaagacaaagcgaagaaccctatacttgaaagtccaagagattctagtgactttacaactcataagaagtttatgttgaacactaatttcaataacaataaagcatcacacatgactatgttggagaatcaagaagctgctgcatttcgtaaaggttggaaagaatatatctgtaatttagaagaaggcgataaggtttacctttatcaaagtggcgttggttttgtagcatctggtattgtcactggtgacttaatcaaaagtgagtatcgtggacaaccagaagaaaaatattctaaaaaattaaaggattttaaaataggatttaaagcaatttctgcaaaagagtttaagaccttaactggcggtggtgctagctttcgtacaacaatgagcgagctaaagcctgaacaatgtagaaaattagatatggaaatagaaaaacggatgaagtcagtaagttaaaaatatgagttgttgttttagtgtgtcacgtagcaatcacttagaagttccctttgtattacttgtctagcaatggttttaaaaagcgtcactactgatagtgacgctttttttgtttttcaaaggaagtaattagcgagtgtctacgagcgacacaatgaaagttcgattattccctcctctaaaaaaccgctt

SEQ ID NO: 47 - DNA, 1328 bp, Artificial Sequence
  source 1..1328: /mol_type="DNA" /note="query" /organism="Artificial Sequence"
ttttaaacctttggacttttcccttaatttgcagaaattgcccctcgactaagcaagcttagtcaaaaaagtttgagcaaagcgaaaacatagggcaattttcatgatgaaaatgggcttttaaagtttttaaatgcttttaaatgcttttagacatgttgaaatgcaagcctagcaaggcatacagaggacatacccctacgtttaccgatcaatacccctacgtttaccgatcaatacccctacgtttaccgatcaatacccctacgtttaccttgcatatcactacaaacaatattaatgtagtaataacttcaaaataataaatgtaggttatgagcgatttaatagtaaaggataacgccctaatgaacgctagttacaacttagctttggttgaacagcgtttaatccttttagctatattggaagcgagagaaacaggaaaagggattaatgccaatgaccccttaacagttcatgcaagtagctatatcaatcaatttaacgtggaaagacatacggcatatcaagcattaaaagatgcttgcaaagacttgtttgcacgtcaatttagttaccaagaaaagcgagaacgaggacgaattaatattacaagtcgatgggtttcacaaattggttatatggacgatacagcaaccgttgaaattatttttgcccctgcggttgttcctttgattacacgtttagaggaacaattcactcaatacgatattgaacaaattagcgagttatcgagtgcttatgctgtccgcctatatgagttactaatttgttggcgtagcacaggaaaaaccccaattattgatctaacagagtttagaaagcgtctaggcgttttagataccgaatacactaggacagataacttgaagatgcgagtgattgagctaggacttaaacaaatcaacgagcatacggacattacagcaagctacgaacagcacaaaaaagggcggacaatcacaggattctcattcaagtttaagcagaagaagaaaacaggggcggaaatgccaaaaaatagcgattctagcccacatatcgaaaaacctagtcaaatccctgccaacatcgcaaaacagcctgaaaatgccaaaaaagatgatttagggcacagagcaagcaagattacagggttaattatgtcgaatggtttagcagatcggtttaaacgtggtgatgagtcagtaatagacatgatgaaacgcatcgaggaaattacaactgatacaacagcagaccaatgggaaaacaagctagaagaatttggcgtgatttttcagtcatgatcaatttcccgaagg

SEQ ID NO: 48 - DNA, 1324 bp, Artificial Sequence; identical to SEQ ID NO: 3
  source 1..1324: /mol_type="DNA" /note="subject" /organism="Artificial Sequence"

SEQ ID NO: 49 - DNA, 91 bp, Artificial Sequence
  source 1..91: /mol_type="DNA" /note="query" /organism="Artificial Sequence"
ttaaaaatattggttgctagatggttttaactatcgtggagcttttgcttttaaaaatacacgaagcaaagcgagttcatagtcgcttttg

SEQ ID NO: 50 - DNA, 89 bp, Artificial Sequence
  source 1..89: /mol_type="DNA" /note="subject" /organism="Artificial Sequence"
ttaaaaatattggctgctagatggtttttactatagtgaggttttgcttttaaaaaaacacgagcaaagcgagttcatagttgcttttg

SEQ ID NO: 51 - DNA, 64 bp, Artificial Sequence
  source 1..64: /mol_type="DNA" /note="query" /organism="Artificial Sequence"
attagcgagtgtctacgagcgacacaatgaaagttcgattattccctcctctaaaaaaccgctt

SEQ ID NO: 52 - DNA, 63 bp, Artificial Sequence
  source 1..63: /mol_type="DNA" /note="subject" /organism="Artificial Sequence"
attagcgagtgtctacgagcgactcaatgaaagttcgattattccccctctggaaaaccgctt

SEQ ID NO: 53 - protein, 304 aa, Artificial Sequence
  SOURCE 1..304: /mol_type="protein" /note="query" /organism="Artificial Sequence"
  VARIANT 301: unknown or other
MSDLIVKDNALMNASYNLALVEQRLILLAILEARETGKGINANDPLTVHASSYINQFNVERHTAYQALKDACKDLFARQFSYQEKRERGRINITSRWVSQIGYMDDTATVEIIFAPAVVPLITRLEEQFTQYDIEQISELSSAYAVRLYELLICWRSTGKTPIIDLTEFRKRLGVLDTEYTRTDNLKMRVIELGLKQINEHTDITASYEQHKKGRTITGFSFKFKQKKKTGAEMPKNSDSSPHIEKPSQIPANIAKQPENAKKDDLGHRASKITGLIMSNGLADRFKRGDESVIDMMKRIXRKL

SEQ ID NO: 54 - protein, 304 aa, Artificial Sequence
  SOURCE 1..304: /mol_type="protein" /note="subject" /organism="Artificial Sequence"
MSDLIVKDNALMNASYNLALVEQRLILLAIIEARETGKGINANDPLTVHAGSYINQFNVQRHTAYQALKDACKDLFARQFSYQEKRERGRINITSRWVSQIGYMDDTATVEIIFAPAVVPLITRLEEQFTQYDIEQISGLSSAYAVRMYELLICWRSTGKTPIIELDEFRKRIGVLDTEYTRTDNLKMQVIELALKQINEHTDITASYEQHKKGRVITGFSFMFKHKKQNSDKTPDTNASSPRIVKHSQIPTNIVKQPENAKMSDLEHRASRVTGEIMRNRLSDRFKQGDESAIDMMKRIQSEI

SEQ ID NO: 55 - protein, 304 aa, Artificial Sequence; identical to SEQ ID NO: 53
  SOURCE 1..304: /mol_type="protein" /note="query" /organism="Artificial Sequence"
  UNSURE 301: unknown or other

SEQ ID NO: 56 - protein, 304 aa, Artificial Sequence
  SOURCE 1..304: /mol_type="protein" /note="subject" /organism="Artificial Sequence"
MSELIVKDNALMNASYNLDLVEQRLILLAIVEARESGKGINANDPLTVHAESYINQFGVHRTTAYQALKDACKDLFARQFSYQEKRERGRANITSRWVSQIAYIDETATVEIIFAPAVVPLITRLEKQFTQYDIEQISGLSSAYAVRMYELLICWRSTGKTPVIELGEFRKRIGVLDTEYIRTDNLKMRVIELALKQINDHTDITATYEQHKKGRTITGFSFKFKQKRKTELETPKNSDSDVPKQKSVEIPTNLVKQPENANMSDLQHRASKITGLIMSNRLSDRFKQSDESIMQMMARIQSEI

SEQ ID NO: 57 - DNA, 2148 bp, Artificial Sequence
  source 1..2148: /mol_type="DNA" /note="CMI2.214" /organism="Artificial Sequence"
ttgtactgaattaatgaacgagtgtctacgagtggcataaagaaagttcgcttattgcccctctgaaaaaccgctttttctatatctaatttcatgaaaattttaactactgtgagcttttgcttttgaaaagacacgagcgaagcgagtgccattttttgctcttgcttttggggtttggggcttgccccaacagggcacagagtaggaattttacacggtagtgaaaaagtcccctctgtgtgtccttgccctatgctttttaaacctttgaatttttccctgtaatttgaagaaattgcccctcgactaagcttgcttagtcaaaaaagtttgagcaaagcgaaaacatagggcaattttcataataaaaatgggcttttaaagtttttaaatgcttttaaatgcttttagacatgctgaaatgcctacacagcaaggcatacagaggacatactcctaggtttacccaccaatactcctaggtttacctaccaatactcctaggtttacctaccaatactcctaggtttaccttgcgtaatcctaaaagatataatacaaaggaactactaggtttaatattaataagtaaaatgagcgatttaatagtaaaagataatgccttaatgaacgctagttataacctagacttagttgagcagcgtttaattctcttggctatccttgaggcgagagaaacaggcaaagggattaatgccaatgatcctctaaccgttcatgctgaaagctatatcaatcaatttggtgtagctagacagactgcatatcaagcattaaaagatgcttgtaaggacttatttgcacgccaatttagttaccaagaaaaacgtgagcgtgggcgagctaatattacaagtcgttgggtatcgcaaattgcttacattgatgaaacggcaacagttgaggttatttttgcccctgccgttgttccactgattacacgattagaggaacaattcacccaatacgatattgaacaaattagcggtttatcgagtgcctatgccgtccgtctatatgaattattgatttgttggcgtagtacagggaaaacacctgttattgaactagcagagtttagaaagcgtttaggtgttttaaatgatgaatatactagatcggataatttcaaaaaatggattattgaaaaccctattaaacaaataaacgagcataccgacatcacagcaagctacgaacagcacaaaaaagggcggacaatcacagggttttcattcaagtttaagcagaagaaaaaaacagaacctgaaacgccaaaaaacagcgattctagccaacgtatcgaaaagcctagtcaaatccctgccaacatcgtaaaacaacctgaaaacgcaaatttgagcgatttacagcatcgagcaagcaagattacagggttaatcatgtctaaccgtctatcagatcggtttaaacaaggtgatgaatcaatcatgcagatgatggcacgtattcaaagtgagattacaaccgattcaatagccgaccaatggcaatcaaaattagaagaatttggcgtagttttttagtctgtcacgtagcaatcacgtagaaaattatgcttgaaaggcttgctgttattacatttcaaaaagcgtcactactgatagtgacgcttttcttagtttgcctgttgaattaaacagtgagtgatagacctcttttggttaggacttcattaaccttttcatgccattctttaattatttttgtcgtttctgcattttcactagaacaaataactaatgtttttcttggctgaggtagtgttttcccccaaatgtcccaatccaatacacgaatagggcgtctgaaaacaatccaatcggtttcactttcatcaccattgacttcataagctccaccaattacctgaactaatgcaattaatttgccaccatttttaatagcaacaatatcattcactttcattctgttaaaaaagtcctctttttcaacctgtcctccagcccattttcctaaacctataatttttttgttctctaaaattgaatgtaaaacttccgaaaagctttgatcatcagggtgcatctgcatatgccaatattgagtcatgttttttttccataggtaattatgtttgtt

SEQ ID NO: 58 - DNA, 960 bp, Artificial Sequence
  source 1..960: /mol_type="DNA" /note="query" /organism="Artificial Sequence"
ataaacgagcataccgacatcacagcaagctacgaacagcacaaaaaagggcggacaatcacagggttttcattcaagtttaagcagaagaaaaaaacagaacctgaaacgccaaaaaacagcgattctagccaacgtatcgaaaagcctagtcaaatccctgccaacatcgtaaaacaacctgaaaacgcaaatttgagcgatttacagcatcgagcaagcaagattacagggttaatcatgtctaaccgtctatcagatcggtttaaacaaggtgatgaatcaatcatgcagatgatggcacgtattcaaagtgagattacaaccgattcaatagccgaccaatggcaatcaaaattagaagaatttggcgtagttttttagtctgtcacgtagcaatcacgtagaaaattatgcttgaaaggcttgctgttattacatttcaaaaagcgtcactactgatagtgacgcttttcttagtttgcctgttgaattaaacagtgagtgatagacctcttttggttaggacttcattaaccttttcatgccattctttaattatttttgtcgtttctgcattttcactagaacaaataactaatgtttttcttggctgaggtagtgttttcccccaaatgtcccaatccaatacacgaatagggcgtctgaaaacaatccaatcggtttcactttcatcaccattgacttcataagctccaccaattacctgaactaatgcaattaatttgccaccatttttaatagcaacaatatcattcactttcattctgttaaaaaagtcctctttttcaacctgtcctccagcccattttcctaaacctataatttttttgttctctaaaattgaatgtaaaacttccgaaaagctttgatcatcagggtgcatctgcatatgccaatattgagtcatgttttttttccataggtaattatgtttgt

SEQ ID NO: 59 - DNA, 959 bp, Artificial Sequence
  source 1..959: /mol_type="DNA" /note="subject" /organism="Artificial Sequence"
ataaacgagtacaccgacatcatagcaagctacgaacagcacaaaaaagggcggacaatcacagggttttcattcaagtttaagcagaagaaaaaaacagaacctgaaacgccaaaaaatagcgattctagccaacgtatcgaaaagcctagtcaaatccctgccaacatcgtaaaacaacctgaaaacgcaaatttgagcgatttacagcatcgagcaagcaagattacagggttaatcatgtctaaccgtctatcagatcggtttaaacaaggtgatgaatcaatcatgcagatgatggcacgtattcaaagtgagattacaaccgattcaatagccgaccaatggcaatcaaaattagaagaatttggcgtagttttttagtctgtcacgtggcaatcacgtagaaaattatgtttgaaaggcttgctgttattacatttcaaaaagcgtcactactgatagtgacgcttttcttagtttgcctgttgaattaaacagtgagtgatagacctctttttgttaggacttcattaaccttttcatgccattctttaattatttttgtcgtttctgcattttcactagaacaaataactaatgtttttcttggctgaggtagtgttttcccccaaatgtcccaatccaatatacgaatagggcgtctgaaaacaatccaatcggtttcactttcatcatcattgacttcataagctccaccaattacctgaactaatgcaattaatttgccaccatttttaatagcaacaatatcattcactttcattctgttagaaaagtcctctttttcaacctgtcctccagcccattttcctaaacctataatttttttgttctctaaaattgaatgtaaaacttctgaaaagttttgatcatcagggtgcatctgcatatgccaatattgagtcatgtttttttccataggtaattatgtttgt

SEQ ID NO: 60 - DNA, 150 bp, Artificial Sequence
  source 1..150: /mol_type="DNA" /note="query" /organism="Artificial Sequence"
ttgtactgaattaatgaacgagtgtctacgagtggcataaagaaagttcgcttattgcccctctgaaaaaccgctttttctatatctaatttcatgaaaattttaactactgtgagcttttgcttttgaaaagacacgagcgaagcgagt

SEQ ID NO: 61 - DNA, 151 bp, Artificial Sequence
  source 1..151: /mol_type="DNA" /note="subject" /organism="Artificial Sequence"
ttgtactgaattaatgaacgagtgtctacgagtggcataaagaaagttcgctcattgccctctttgaaaaaccgcttttaaaaatactggctgctcgataatttttactatcgagtgcttttgcttttgaaaaaatacgagcgaagcgagt

SEQ ID NO: 62 - DNA, 48 bp, Artificial Sequence
  source 1..48: /mol_type="DNA" /note="query" /organism="Artificial Sequence"
ataaacgagcataccgacatcacagcaagctacgaacagcacaaaaaa

SEQ ID NO: 63 - DNA, 48 bp, Artificial Sequence
  source 1..48: /mol_type="DNA" /note="subject" /organism="Artificial Sequence"
ataaacgagtacaccgacatcacagccacctacgaacagcacaaaaaa

SEQ ID NO: 64 - DNA, 1607 bp, Artificial Sequence
  source 1..1607: /mol_type="DNA" /note="query" /organism="Artificial Sequence"
cgagtgtctacgagtggcataaagaaagttcgcttattgcccctctgaaaaaccgctttttctatatctaatttcatgaaaattttaactactgtgagcttttgcttttgaaaagacacgagcgaagcgagtgccattttttgctcttgcttttggggtttggggcttgccccaacagggcacagagtaggaattttacacggtagtgaaaaagtcccctctgtgtgtaacaagtcctcgaatatcaaaatgtggctacattttgtatatacgggtaggcttgcttatttgattttttttcttctaaacctttgacttcttccccattgtttgcagaaattgcccctcgaagcttgcttagtcaaaaaagtttgagcaaagcgaaaacatagggcaattttcatgaagaaattgggcttttaaagtttttaaatgttttaaatgcttttagacatgctaagaagcccacacagcaaggcatacagaggacattctcctacgtttaccgatcaatacccccgtttaccgatcaatacccctacgtttaccgatcaatacccctacgtttaccttgcgtataactacaaagaatactagtgtagtataacttcaaaagaataattgtaggttatgagcgatttaatagtaaaagataacgccctaatgaatgctagttataacttagctttggttgaacagaggttaattctattagcaatcatagaagcgagagaaacaggcaaagggattaatgccaatgatcctcttacggttcatgcaggtagctatatcaatcaatttaacgtacaaaggcatacggcatatcaagccctcaaagatgcttgtaaagacttgtttgcccgtcaattcagttaccaagaaaagcgagaacgaggacgaattaatattacaagtcgatgggtttcgcaaattggctatatggacgatacagcaaccgttgagattatttttgcccctgcggttgttcctctgattacacggctagaggaacagttcacccagtacgatattgagcaaattagcggtttatcgagtgcatatgctgttcgtatgtacgaactgctgatttgttggcgtagcacaggcaaaacaccaattattgagctagacgagtttagaaagcgaataggtgttttagatactgaatacactagaacagataatttaaagatgcaagttattgaattagccctaaaacaaatcaacgaacatactgacatcacagcaagctatgaacaacacaaaaaagggcgagtgattaccggattctcattcatgtttaagcacaagaaacaaaacagcgataaaacgcctgatactaacgcttctagcccacgtatcgtaaaacatagtcaaatccctaccaacattgtaaaacagcctgaaaacgccaaaatgagcgatttagaacatagagcgagccgtgttacaggggaaataatgcgaaatcgtctgtcagatcggtttaaacaaggcgatgaatcagcaatcgacatgatgaaacgtattcaaagtgaaataataaccgatgcaatagcagaccagtgggaaagcaaactggaggagtttggcgtggttttttagtc

SEQ ID NO: 65 - DNA, 1556 bp, Artificial Sequence
  source 1..1556: /mol_type="DNA" /note="subject" /organism="Artificial Sequence"
cgagtgtctacgagcgactcaatgaaagttcgattattccccctctggaaaaccgcttttaaaaatattggctgctagatggtttttactatagtgaggttttgcttttaaaaaaacacgagcaaagcgagttcatagttgcttttgcttgttttcgggtcttaggggaaatcccctaacaagtcctcgaatatcaaaatgtggctacattttgtatatacgggtaggcttgcttatttgattttttttcttctaaacctttgacttcttccccattgtttgcagaaattgcccctcgaagcttgcttagtcaaaaaagtttgagcaaagcgaaaacatagggcaattttcatgaagaaattgggcttttaaagtttttaaatgttttaaatgcttttagacatgctaagaagcccacacagcaaggcatacagaggacattctcctacgtttaccgatcaatacccccgtttaccgatcaatacccctacgtttaccgatcaatacccctacgtttaccttgcgtataactacaaagaatactagtgtagtataacttcaaaagaataattgtaggttatgagcgatttaatagtaaaagataacgccctaatgaatgctagttataacttagctttggttgaacagaggttaattctattagcaatcatagaagcgagagaaacaggcaaagggattaatgccaatgatcctcttacggttcatgcaggtagctatatcaatcaatttaacgtacaaaggcatacggcatatcaagccctcaaagatgcttgtaaagacttgtttgcccgtcaattcagttaccaagaaaagcgagaacgaggacgaattaatattacaagtcgatgggtttcgcaaattggctatatggacgatacagcaaccgttgagattatttttgcccctgcggttgttcctctgattacacggctagaggaacagttcacccagtacgatattgagcaaattagcggtttatcgagtgcatatgctgttcgtatgtacgaactgctgatttgttggcgtagcacaggcaaaacaccaattattgagctagacgagtttagaaagcgaataggtgttttagatactgaatacactagaacagataatttaaagatgcaagttattgaattagccctaaaacaaatcaacgaacatactgacatcacagcaagctatgaacaacacaaaaaagggcgagtgattaccggattctcattcatgtttaagcacaagaaacaaaacagcgataaaacgcctgatactaacgcttctagcccacgtatcgtaaaacatagtcaaatccctaccaacattgtaaaacagcctgaaaacgccaaaatgagcgatttagaacatagagcgagccgtgttacaggggaaataatgcgaaatcgtctgtcagatcggtttaaacaaggcgatgaatcagcaatcgacatgatgaaacgtattcaaagtgaaataataaccgatgcaatagcagaccagtgggaaagcaaactggaggagtttggcgtggttttttagtc

SEQ ID NO: 66 - protein, 324 aa, Artificial Sequence
  SOURCE 1..324: /mol_type="protein" /note="query" /organism="Artificial Sequence"
MSDLIVKDNALMNASYNLDLVEQRLILLAILEARETGKGINANDPLTVHAESYINQFGVARQTAYQALKDACKDLFARQFSYQEKRERGRANITSRWVSQIAYIDETATVEVIFAPAVVPLITRLEEQFTQYDIEQISGLSSAYAVRLYELLICWRSTGKTPVIELAEFRKRLGVLNDEYTRSDNFKKWIIENPIKQINEHTDITASYEQHKKGRTITGFSFKFKQKKKTEPETPKNSDSSQRIEKPSQIPANIVKQPENANLSDLQHRASKITGLIMSNRLSDRFKQGDESIMQMMARIQSEITTDSIADQWQSKLEEFGVVF

SEQ ID NO: 67 - protein, 324 aa, Artificial Sequence; identical to SEQ ID NO: 9
  SOURCE 1..324: /mol_type="protein" /note="subject" /organism="Artificial Sequence"

SEQ ID NO: 68 - protein, 324 aa, Artificial Sequence; identical to SEQ ID NO: 66
  SOURCE 1..324: /mol_type="protein" /note="query" /organism="Artificial Sequence"

SEQ ID NO: 69 - protein, 324 aa, Artificial Sequence; identical to SEQ ID NO: 7
  SOURCE 1..324: /mol_type="protein" /note="subject" /organism="Artificial Sequence"

SEQ ID NO: 70 - DNA, 1687 bp, Artificial Sequence
  source 1..1687: /mol_type="DNA" /note="CMI3.168" /organism="Artificial Sequence"
ggattaatgccaatgatcccttaacagttcatgcaagtagctatatcaatcaatttaacgttgaaagacatacggcatatcaagcattaaaagatgcttgtaaggacttatttgcacgccaatttagttaccaagaaaaacgtgagcgtgggcgagctaatattacaagtcgttgggtatcgcaaattgcttacattgatgaaacggcaacagttgaggttatttttgcccctgccgttgttccactgattacacgattagaggaacaattcacccaatacgatattgaacaaattagcggtttatcgagtgcctatgcagttcgcttatatgagttattgatctgctggagaacaacaggaaagacaccagttcttgacttaacagagtttagaaagcgtctaggtgttttagataccgaatacactagaacagataacttgaagatgcgagtgattgagcagtcactcaagcaaataaacaagcataccgacatcacagcgagctacgaacagcacaaaaaagggcggacaatcacaggattctcattcaagtttaagcagaagaagaaaacagagccagaaacgccaaaaaacaacgattctggcgtttctaagccgaaaacagtagaaatccctgccgaagtcgtaaaacagcctaaaaacaccaatttgagcgatttagagaaacgagtaaggatgatcacaggggcaattgctaaaaataacctggcaagtcgttttcaacatgggaatgaatcaccactggatatgatgaaacgtattcaaagtgaaatcacatcagacgaaactgccgatctatggcaaaacaaacttgaatcaatgggtgtggttttttagtcatgacgaatttcccgaagggcgcactttcccaaactatcgtttgagtgcgtttttctatcgaaaaagtaaaaagacaaagaaaattttctttgtctttttttctgtttttcaaaaaaagggattagcgagtgtctacgagcgacacaatgaaagttcgattatttccccctctgaaaaaccgcttttttgtatctgatttcaagaaaattttaactatcgtgcgcttttgcttttgagaagacacgagcgaagcgagtgccatttttgcctttgcttttgctttttggggtttggggcttgccccaacaaggcacagagtaggaattttacacggtagtggaaaagtcccctctgtgtgtccttgctctaatctttttaaaacctttgattcttcaccgtaatttgctaaaaattgccccgactgagtgaagcgaagtcaaaaaagtttgagcaaagcgaaaacatagggcaattttcgtgatgaaaatgggcttttaaggtttttaaatgcttttaaatgcttttagacacgctgaaacgcaagcctagcaaggtatacagagggcatttacctacgtttaccgatcaatacccctacgtttaccgatcaatacccctacgtttaccgatcaatacccctacgtttaccttgcatataactacaaaatataataatgtagtaataacttcaaaataataaacgtaggttatgagcgatttaatagtaaaagataacgccctaatgaacgctagttacaacttagctttggttgaacagcgtttaattctattggctatcctagaggcgagagaaacaggcaaag

SEQ ID NO: 71 - DNA, 22 bp, Artificial Sequence
  source 1..22: /mol_type="DNA" /note="repeat" /organism="Artificial Sequence"
atacccctacgtttaccgatca

SEQ ID NO: 72 - DNA, 889 bp, Artificial Sequence
  source 1..889: /mol_type="DNA" /note="query" /organism="Artificial Sequence"
ggattaatgccaatgatcccttaacagttcatgcaagtagctatatcaatcaatttaacgttgaaagacatacggcatatcaagcattaaaagatgcttgtaaggacttatttgcacgccaatttagttaccaagaaaaacgtgagcgtgggcgagctaatattacaagtcgttgggtatcgcaaattgcttacattgatgaaacggcaacagttgaggttatttttgcccctgccgttgttccactgattacacgattagaggaacaattcacccaatacgatattgaacaaattagcggtttatcgagtgcctatgcagttcgcttatatgagttattgatctgctggagaacaacaggaaagacaccagttcttgacttaacagagtttagaaagcgtctaggtgttttagataccgaatacactagaacagataacttgaagatgcgagtgattgagcagtcactcaagcaaataaacaagcataccgacatcacagcgagctacgaacagcacaaaaaagggcggacaatcacaggattctcattcaagtttaagcagaagaagaaaacagagccagaaacgccaaaaaacaacgattctggcgtttctaagccgaaaacagtagaaatccctgccgaagtcgtaaaacagcctaaaaacaccaatttgagcgatttagagaaacgagtaaggatgatcacaggggcaattgctaaaaataacctggcaagtcgttttcaacatgggaatgaatcaccactggatatgatgaaacgtattcaaagtgaaatcacatcagacgaaactgccgatctatggcaaaacaaacttgaatcaatgggtgtggttttttagtcatgacgaatttcccgaagggcgcactt

SEQ ID NO: 73 - DNA, 888 bp, Artificial Sequence
  source 1..888: /mol_type="DNA" /note="subject" /organism="Artificial Sequence"
ggattaatgccaatgatcctcttacggttcatgcaggtagctatatcaatcaatttaacgtacaaaggcatacggcatatcaagccctcaaagatgcttgtaaagacttgtttgcccgtcaattcagttaccaagaaaagcgagaacgaggacgaattaatattacaagtcgatgggtttcgcaaattggctatatggacgatacagcaaccgttgagattatttttgcccctgcggttgttcctctgattacacggctagaggaacagttcacccagtacgatattgagcaaattagcggtttatcgagtgcatatgctgttcgtatgtacgaactgctgatttgttggcgtagcacaggcaaaacaccaattattgagctagacgagtttagaaagcgaataggtgttttagatactgaatacactagaacagataatttaaagatgcaagttattgaattagccctaaaacaaatcaacgaacatactgacatcacagcaagctatgaacaacacaaaaaagggcgagtgattaccggattctcattcatgtttaagcacaagaaacaaaacagcgataaaacgcctgatactaacgcttctagcccacgtatcgtaaaacatagtcaaatccctaccaacattgtaaaacagcctgaaaacgccaaaatgagcgatttagaacatagagcgagccgtgttacaggggaaataatgcgaaatcgtctgtcagatcggtttaaacaaggcgatgaatcagcaatcgacatgatgaaacgtattcaaagtgaaataataaccgatgcaatagcagaccagtgggaaagcaaactggaggagtttggcgtggttttttagtcatgacgatttcccgaagggcgcactt

SEQ ID NO: 74 - DNA, 717 bp, Artificial Sequence
  source 1..717: /mol_type="DNA" /note="query" /organism="Artificial Sequence"
ttcaaaaaaagggattagcgagtgtctacgagcgacacaatgaaagttcgattatttccccctctgaaaaaccgcttttttgtatctgatttcaagaaaattttaactatcgtgcgcttttgcttttgagaagacacgagcgaagcgagtgccatttttgcctttgcttttgctttttggggtttggggcttgccccaacaaggcacagagtaggaattttacacggtagtggaaaagtcccctctgtgtgtccttgctctaatctttttaaaacctttgattcttcaccgtaatttgctaaaaattgccccgactgagtgaagcgaagtcaaaaaagtttgagcaaagcgaaaacatagggcaattttcgtgatgaaaatgggcttttaaggtttttaaatgcttttaaatgcttttagacacgctgaaacgcaagcctagcaaggtatacagagggcatttacctacgtttaccgatcaatacccctacgtttaccgatcaatacccctacgtttaccgatcaatacccctacgtttaccttgcatataactacaaaatataataatgtagtaataacttcaaaataataaacgtaggttatgagcgatttaatagtaaaagataacgccctaatgaacgctagttacaacttagctttggttgaacagcgtttaattctattggctatcctagaggcgagagaaacaggcaaag

SEQ ID NO: 75 - DNA, 713 bp, Artificial Sequence
  source 1..713: /mol_type="DNA" /note="subject" /organism="Artificial Sequence"
ttcacaaaaaagatattagcgagtgtctacgagcgactcaatgaaagttcgattattccccctctggaaaaccgcttttaaaaatattggctgctagatggtttttactatagtgaggttttgcttttaaaaaaacacgagcaaagcgagttcatagttgcttttgcttgttttcgggtcttaggggaaatcccctaacaagtcctcgaatatcaaaatgtggctacattttgtatatacgggtaggcttgcttatttgattttttttcttctaaacctttgacttcttccccattgtttgcagaaattgcccctcgaagcttgcttagtcaaaaaagtttgagcaaagcgaaaacatagggcaattttcatgaagaaattgggcttttaaagtttttaaatgttttaaatgcttttagacatgctaagaagcccacacagcaaggcatacagaggacattctcctacgtttaccgatcaatacccccgtttaccgatcaatacccctacgtttaccgatcaatacccctacgtttaccttgcgtataactacaaagaatactagtgtagtataacttcaaaagaataattgtaggttatgagcgatttaatagtaaaagataacgccctaatgaatgctagttataacttagctttggttgaacagaggttaattctattagcaatcatagaagcgagagaaacaggcaaag

SEQ ID NO: 76 - protein, 324 aa, Artificial Sequence
  SOURCE 1..324: /mol_type="protein" /note="query" /organism="Artificial Sequence"
MSDLIVKDNALMNASYNLALVEQRLILLAILEARETGKGINANDPLTVHASSYINQFNVERHTAYQALKDACKDLFARQFSYQEKRERGRANITSRWVSQIAYIDETATVEVIFAPAVVPLITRLEEQFTQYDIEQISGLSSAYAVRLYELLICWRTTGKTPVLDLTEFRKRLGVLDTEYTRTDNLKMRVIEQSLKQINKHTDITASYEQHKKGRTITGFSFKFKQKKKTEPETPKNNDSGVSKPKTVEIPAEVVKQPKNTNLSDLEKRVRMITGAIAKNNLASRFQHGNESPLDMMKRIQSEITSDETADLWQNKLESMGVVF

SEQ ID NO: 77 - protein, 324 aa, Artificial Sequence; identical to SEQ ID NO: 9
  SOURCE 1..324: /mol_type="protein" /note="subject" /organism="Artificial Sequence"

SEQ ID NO: 78 - protein, 264 aa, Artificial Sequence
  SOURCE 1..264: /mol_type="protein" /note="query" /organism="Artificial Sequence"
MSDLIVKDNALMNASYNLALVEQRLILLAILEARETGKGINANDPLTVHASSYINQFNVERHTAYQALKDACKDLFARQFSYQEKRERGRANITSRWVSQIAYIDETATVEVIFAPAVVPLITRLEEQFTQYDIEQISGLSSAYAVRLYELLICWRTTGKTPVLDLTEFRKRLGVLDTEYTRTDNLKMRVIEQSLKQINKHTDITASYEQHKKGRTITGFSFKFKQKKKTEPETPKNNDSQSEITSDETADLWQNKLESMGVVF

SEQ ID NO: 79 - protein, 324 aa, Artificial Sequence; identical to SEQ ID NO: 7
  SOURCE 1..324: /mol_type="protein" /note="subject" /organism="Artificial Sequence"

SEQ ID NO: 80 - protein, 137 aa, Artificial Sequence
  SOURCE 1..137: /mol_type="protein" /note="query" /organism="Artificial Sequence"
MRVIEQSLKQINKHTDITASYEQHKKGRTITGFSFKFKQKKKTEPETPKNNDSGVSKPKTVEIPAEVVKQPKNTNLSDLEKRVRMITGAIAKNNLASRFQHGNESPLDMMKRIQSEITSDETADLWQNKLESMGVVF

SEQ ID NO: 81 - protein, 137 aa, Artificial Sequence
  SOURCE 1..137: /mol_type="protein" /note="subject" /organism="Artificial Sequence"
MRVIELALKQINDHTDITATYEQHKKGRTITGFSFKFKQKRKTELETPKNSDSDVPKQKSVEIPTNLVKQPENANMSDLQHRASKITGLIMSNRLSDRFKQSDESIMQMMARIQSEITDEAIANQWENKLEEFGVIF

SEQ ID NO: 82 - protein, 137 aa, Artificial Sequence; identical to SEQ ID NO: 80
  SOURCE 1..137: /mol_type="protein" /note="query" /organism="Artificial Sequence"

SEQ ID NO: 83 - protein, 137 aa, Artificial Sequence
  SOURCE 1..137: /mol_type="protein" /note="subject" /organism="Artificial Sequence"
MRVIELALKQINDYTDITASYEQHKKGRVITGFSFKFKQKKKTEAETPKNSDSGVSKQKPIEIPTEVVKQPKNANLSDLEHRASRITGEIMRNRLTDRFKQADESPLEMMKRIQSEITTDTIADQWENKLEEFGVVF

SEQ ID NO: 84 - protein, 137 aa, Artificial Sequence; identical to SEQ ID NO: 80
  SOURCE 1..137: /mol_type="protein" /note="query" /organism="Artificial Sequence"

SEQ ID NO: 85 - protein, 137 aa, Artificial Sequence; identical to SEQ ID NO: 83
  SOURCE 1..137: /mol_type="protein" /note="subject" /organism="Artificial Sequence"

SEQ ID NO: 86 - protein, 137 aa, Artificial Sequence; identical to SEQ ID NO: 80
  SOURCE 1..137: /mol_type="protein" /note="query" /organism="Artificial Sequence"

SEQ ID NO: 87 - protein, 137 aa, Artificial Sequence; identical to SEQ ID NO: 83
  SOURCE 1..137: /mol_type="protein" /note="subject" /organism="Artificial Sequence"

SEQ ID NO: 88 - protein, 137 aa, Artificial Sequence; identical to SEQ ID NO: 80
  SOURCE 1..137: /mol_type="protein" /note="query" /organism="Artificial Sequence"

SEQ ID NO: 89 - protein, 137 aa, Artificial Sequence
  SOURCE 1..137: /mol_type="protein" /note="subject" /organism="Artificial Sequence"
MQVIELALKQINEHTDITASYEQHKKGRVITGFSFMFKHKKQNSDKTPDTNASSPRIVKHSQIPTNIVKQPENAKMSDLEHRASRVTGEIMRNRLSDRFKQGDESAIDMMKRIQSEIITDAIADQWESKLEEFGVVF

SEQ ID NO: 90 - DNA, 1583 bp, Artificial Sequence
  source 1..1583: /mol_type="DNA" /note="CMI4.158" /organism="Artificial Sequence"
gaggacgaattaatattacaagtcgttgggtttcacaaattggttatatggacgatacagcaaccgttgaggttatttttgcccctgcggttgttccattgattacaagactggaggaacaattcacccagtacgatattgagcaaattagcggtttatctagtgcttatgccgtccgtctgtatgaattattgatctgttggcgtagcacaggaaaaacgcccgtcatagaactagcagagtttagaaaacgaataggtgttttagatactgaatacacgagaacagataacttaaagatgcgagttattgagctagcactcaagcagatcaacgaacatacagacatcacagcaagctatgaacagcacaaaaaagggcggacaatcactgggttctcattcaagtttaagcagaagaagaaaacagagctagaaacgccaaaaaacagcgattctagcccacatatcgaaaaacctagtcaaatccctaccaacatcgtaaaacagcctgaaaacgccaaaaaagacgatttagggcatagagcaagtaagattacaggtttaatcatgtccaatggtttagcagatcggtttaaacgtggtgatgagtccgtcatgaatatgatgaaacgcatcaaagaagaaattacaaccgatgcaacagccgatctatggcaaaacaaacttgaatcaatggtgtggttttttagtcatgactaaattggctatgcaatgtctccgctctttttctaagaaccgtttttgctttttcaaaatcgcggctcgcgggtgtctttactggtatatgcgctttttcgtgctgcttttcaaaaaatgtggcgatagccaacattctcgattttgatcttgattttggggttttagggtctccctaacaagacatagagacacaactcgctagaggggtctctatgtgtccttgcccttaattaaaaaactaaataaatttttacccgtttttgctttaaaaaaggcaggtttttctttgtccttacttttgactttgattttctcctgtttttttgagttacccacaagaattttcatgtggttttgggcttttaaggtttttaaatgcttttaaatgcttttaaacatgctgaaacgtaagcatagcaaggtatacagagttcattctcctacgtttaccgatcaatacccctacgtttaccgatcaatacccctacgtttaccgatcaatacccctacgtttaccgatcaatacccctacgtttaccttgcatataactacaaaaaacaataatgtagtaataacttcaaaataataagagtaggttatgagcgatttaatagtaaaagataacgccctaatgaacgctagttacaacttagctttggttgaacagcgtttaattcttttagctatattggaagcgagagaaacaggaaaagggattaatgccaatgatcccttaacagttcatgcaaatagctatatcaatcaatttaacgtggaaagacatacggcatatcaagcattaaaagatgcctgcaaagacttgtttgcacgtcaattcagttaccaagaaaagcgagaac

SEQ ID NO: 91 - DNA, 1002 bp, Artificial Sequence
  source 1..1002: /mol_type="DNA" /note="query" /organism="Artificial Sequence"
tcaaaataataagagtaggttatgagcgatttaatagtaaaagataacgccctaatgaacgctagttacaacttagctttggttgaacagcgtttaattcttttagctatattggaagcgagagaaacaggaaaagggattaatgccaatgatcccttaacagttcatgcaaatagctatatcaatcaatttaacgtggaaagacatacggcatatcaagcattaaaagatgcctgcaaagacttgtttgcacgtcaattcagttaccaagaaaagcgagaacgaggacgaattaatattacaagtcgttgggtttcacaaattggttatatggacgatacagcaaccgttgaggttatttttgcccctgcggttgttccattgattacaagactggaggaacaattcacccagtacgatattgagcaaattagcggtttatctagtgcttatgccgtccgtctgtatgaattattgatctgttggcgtagcacaggaaaaacgcccgtcatagaactagcagagtttagaaaacgaataggtgttttagatactgaatacacgagaacagataacttaaagatgcgagttattgagctagcactcaagcagatcaacgaacatacagacatcacagcaagctatgaacagcacaaaaaagggcggacaatcactgggttctcattcaagtttaagcagaagaagaaaacagagctagaaacgccaaaaaacagcgattctagcccacatatcgaaaaacctagtcaaatccctaccaacatcgtaaaacagcctgaaaacgccaaaaaagacgatttagggcatagagcaagtaagattacaggtttaatcatgtccaatggtttagcagatcggtttaaacgtggtgatgagtccgtcatgaatatgatgaaacgcatcaaagaagaaattacaaccgatgcaacagccgatctatggcaaaacaaacttgaatcaatggtgtggttttttagtcatgac

SEQ ID NO: 92 - DNA, 1003 bp, Artificial Sequence
  source 1..1003: /mol_type="DNA" /note="subject" /organism="Artificial Sequence"
tcaaaagaataattgtaggttatgagcgatttaatagtaaaagataacgccctaatgaatgctagttataacttagctttggttgaacagaggttaattctattagcaatcatagaagcgagagaaacaggcaaagggattaatgccaatgatcctcttacggttcatgcaggtagctatatcaatcaatttaacgtacaaaggcatacggcatatcaagccctcaaagatgcttgtaaagacttgtttgcccgtcaattcagttaccaagaaaagcgagaacgaggacgaattaatattacaagtcgatgggtttcgcaaattggctatatggacgatacagcaaccgttgagattatttttgcccctgcggttgttcctctgattacacggctagaggaacagttcacccagtacgatattgagcaaattagcggtttatcgagtgcatatgctgttcgtatgtacgaactgctgatttgttggcgtagcacaggcaaaacaccaattattgagctagacgagtttagaaagcgaataggtgttttagatactgaatacactagaacagataatttaaagatgcaagttattgaattagccctaaaacaaatcaacgaacatactgacatcacagcaagctatgaacaacacaaaaaagggcgagtgattaccggattctcattcatgtttaagcacaagaaacaaaacagcgataaaacgcctgatactaacgcttctagcccacgtatcgtaaaacatagtcaaatccctaccaacattgtaaaacagcctgaaaacgccaaaatgagcgatttagaacatagagcgagccgtgttacaggggaaataatgcgaaatcgtctgtcagatcggtttaaacaaggcgatgaatcagcaatcgacatgatgaaacgtattcaaagtgaaataataaccgatgcaatagcagaccagtgggaaagcaaactggaggagtttggcgtggttttttagtcatgac

SEQ ID NO: 93 - DNA, 178 bp, Artificial Sequence
  source 1..178: /mol_type="DNA" /note="query" /organism="Artificial Sequence"
aattttcatgtggttttgggcttttaaggtttttaaatgcttttaaatgcttttaaacatgctgaaacgtaagcatagcaaggtatacagagttcattctcctacgtttaccgatcaatacccctacgtttaccgatcaatacccctacgtttaccgatcaatacccctacgtttacc

SEQ ID NO: 94 - DNA, 176 bp, Artificial Sequence
  source 1..176: /mol_type="DNA" /note="subject" /organism="Artificial Sequence"
aattttcatgaagaaattgggcttttaaagtttttaaatgttttaaatgcttttagacatgctaagaagcccacacagcaaggcatacagaggacattctcctacgtttaccgatcaatacccccgtttaccgatcaatacccctacgtttaccgatcaatacccctacgtttacc

SEQ ID NO: 95 - protein, 324 aa, Artificial Sequence
  SOURCE 1..324: /mol_type="protein" /note="query" /organism="Artificial Sequence"
MSDLIVKDNALMNASYNLALVEQRLILLAILEARETGKGINANDPLTVHANSYINQFNVERHTAYQALKDACKDLFARQFSYQEKRERGRINITSRWVSQIGYMDDTATVEVIFAPAVVPLITRLEEQFTQYDIEQISGLSSAYAVRLYELLICWRSTGKTPVIELAEFRKRIGVLDTEYTRTDNLKMRVIELALKQINEHTDITASYEQHKKGRTITGFSFKFKQKKKTELETPKNSDSSPHIEKPSQIPTNIVKQPENAKKDDLGHRASKITGLIMSNGLADRFKRGDESVMNMMKRIKEEITTDATADLWQNKLESMVWFF

SEQ ID NO: 96 - protein, 324 aa, Artificial Sequence; identical to SEQ ID NO: 7
  SOURCE 1..324: /mol_type="protein" /note="subject" /organism="Artificial Sequence"

SEQ ID NO: 97 - protein, 324 aa, Artificial Sequence; identical to SEQ ID NO: 95
  SOURCE 1..324: /mol_type="protein" /note="query" /organism="Artificial Sequence"

SEQ ID NO: 98 - protein, 324 aa, Artificial Sequence; identical to SEQ ID NO: 9
  SOURCE 1..324: /mol_type="protein" /note="subject" /organism="Artificial Sequence"

SEQ ID NO: 99 - DNA, 2280 bp, Artificial Sequence
  source 1..2280: /mol_type="DNA" /note="HCBI7.228" /organism="Artificial Sequence"
ctaaggcagatcaacacagggatagaataacacgttttgggattttgaaacatagagcgaagctacaagaacaatatttgtggacgcaggttgatttcaaatctgaaggcgaagacgatctatccaataaggctcttaaggctgcaacaaaattaaaaggttgtggccagtttcttatattcagaaattactacactatcgaccaagttaagctcgaaaaattccacgtatgtggacagcatttgctatgcccaatgtgtgcaggtattcgcgctgctcgctcaatgaaacgctatttagatcgtatccatgaattaatgcgtcagaatccgcgtttaaagcctgttttgatcactttaacggtcaagaacggggaagacttagaagaacgctataatcaccttacaagctcatttagaaagcttctatcgcgttatagggattacaagaaaaagggttgggggtttaaccaattctgtaaaattgatggtgctttctataccactgaatacacctacaacgaaaagacaaaacaatggcatccgcatattcatattttcgctttactcaatgaatggatagaccaggaagaattatctgagacctggcatgacattaccctggattcttatatcatcgatattcgtagagttaaaaaaaccaaagaacacggctatagcaaagctgttgctgaggtatgtaaatacgctcttaagtttggcgatctatcagttgaaaacacttgggatgcatttttaacgcttaagggtaaacgtcttacaggctctttcggttctatgcatggagttaaaattccagataaggccacggatgatatgccactggaggagctgccgtacttagaaatgttctatcgtttcgtgtttgataaaaaatcctactacaacctagaaataacaaaagacgtaacgccacaaacgaattctcgacagagtgaggaggcggcaccaacgaccgacacgactggagagaatgagttgaaggcgcaggatgaagcgaggacgttgccggtgcgagggcacgcagtcacggaacgaccgcagcaagtccatgaatattttgacccatttgatattgagagagaagaatacgacttctacccttaaggggttcgaccccttaaaccccaaagggcgcacttatgcaaacttttcaagttcgccagtgctcccaccagtaacagagggcgcggagtgcgcccgaactgacatcatctaaatttcaaaaccttctctccctgattacaagctcccttttgcctttctccggaaagttttagccatcccaaacgggtggcgacgcattgacaattataatttaatctgcaatattcatcggacattcataaataatctgattggaatattaaatatgctttttaaatctctaggcgttgcaatcgctacaaataatgcttctaactctgacgaagacttgaaaccaattactatccgtttagctgatagtgaaattcaggcgtatgacactgttgcaaaatcaatgggtctaactcgtcaagattttctatcacacgttattcgttccaacttccgacaggctttaaaagagtttgtagtgggttatacaagttcaaatccttctacacccttatctgttttgtttaattcaaatacggacaatgacgaagttaagctcaaactttccaaccttctctcatctatttctcaagaattaatggacgaagaagaaaaagaaattcatgaagcaatcgaaaaccatatgaatacttcctatgcatatgcaactcgtccaaaaggcatctttgttgagaaggatgattcaaaatgattaagcttgaagggatcgttttaaacgtatttacccagcaaggtggtaaagataaaaaaacaggtgatcaatttgctgaccgtgacaaggtgcaaattttaggtgctatggatctgcctaacggtgacgttaaaaatgagttatttacgttatctgtagaaaactatcgggactttaaagacttcttaaatcagaaaatctgtattgctgttggtgcaatggcaagtggtcgcaatgttattttttacgttgctaaaggcgcaaagcctgttttagcagaaatgatgtgaaacacgaaaaaaaacagtgggttagccttggcttctcgctgttttttctttctcttgatactattaactaaagtggggatgaaattgactaaaaaagacaataaaaaagcccataattctgacactttggcgggtgatgaattacaggctttgcaatctg

SEQ ID NO: 100 - DNA, 874 bp, Artificial Sequence
  source 1..874: /mol_type="DNA" /note="query" /organism="Artificial Sequence"
caagaacaatatttgtggacgcaggttgatttcaaatctgaaggcgaagacgatctatccaataaggctcttaaggctgcaacaaaattaaaaggttgtggccagtttcttatattcagaaattactacactatcgaccaagttaagctcgaaaaattccacgtatgtggacagcatttgctatgcccaatgtgtgcaggtattcgcgctgctcgctcaatgaaacgctatttagatcgtatccatgaattaatgcgtcagaatccgcgtttaaagcctgttttgatcactttaacggtcaagaacggggaagacttagaagaacgctataatcaccttacaagctcatttagaaagcttctatcgcgttatagggattacaagaaaaagggttgggggtttaaccaattctgtaaaattgatggtgctttctataccactgaatacacctacaacgaaaagacaaaacaatggcatccgcatattcatattttcgctttactcaatgaatggatagaccaggaagaattatctgagacctggcatgacattaccctggattcttatatcatcgatattcgtagagttaaaaaaaccaaagaacacggctatagcaaagctgttgctgaggtatgtaaatacgctcttaagtttggcgatctatcagttgaaaacacttgggatgcatttttaacgcttaagggtaaacgtcttacaggctctttcggttctatgcatggagttaaaattccagataaggccacggatgatatgccactggaggagctgccgtacttagaaatgttctatcgtttcgtgtttgataaaaaatcctactacaacctagaaataacaaaagacgtaacgccacaaa

SEQ ID NO: 101 - DNA, 871 bp, Artificial Sequence
  source 1..871: /mol_type="DNA" /note="subject" /organism="Artificial Sequence"
caagaacaatatttgtggactcaggttgatttcaaggttggaagtgaaacatctatcaaagctcttaaggctgcaaccaaattaaagggatgcggtcaatttctgctttttcgtaattactacaccatagatcaaatcaagctcgaaaaattccacgtatgcggacagcatttgctatgtccaatgtgtgctggtattcgtgctgcccgttcaatgaatcggtatattcaacgcatcgaagaaataatgcgtcagaatcgcaagctaaagcccgtattgatcactttgaccgttaagaacggtgaagacctacaggaacgctttgaacacctcacaggctcatttaagacgcttttacagcgttaccgtgattttaagaaaaagggtcgagggtttaatcaattttgcaaaattgatggcggtttttatacgaccgaatacacctacaacgaaacaacccaacaatggcatccgcatattcatatttttgcgttagtgactgaccggattgaccaggaggaactagcagaaacttggcacgatataacgcttgattcatacattgtggacatccgcagggtcaaaaaaactaaagaacacggatatgcaaaggctgttgccgaagtctgcaaatacgctcttaagtttagcgatctatccactgagaaaacctttcaagcattttttgacccttaagggcaaaaggcttacaggttcattcggctctatgcatggtgtaaaaattcctgaaagcggacccgatgaaatgcctaaagaggaacttccatatcttgagctgctctatcgtttcgtttttggtgaaaggtcttattacaacctagagttaactaaggacgtaaagccgaacaaa

SEQ ID NO: 102 - DNA, 370 bp, Artificial Sequence
  source 1..370: /mol_type="DNA" /note="query" /organism="Artificial Sequence"
cgtgacaaggtgcaaattttaggtgctatggatctgcctaacggtgacgttaaaaatgagttatttacgttatctgtagaaaactatcgggactttaaagacttcttaaatcagaaaatctgtattgctgttggtgcaatggcaagtggtcgcaatgttattttttacgttgctaaaggcgcaaagcctgttttagcagaaatgatgtgaaacacgaaaaaaaacagtgggttagccttggcttctcgctgttttttctttctcttgatactattaactaaagtggggatgaaattgactaaaaaagacaataaaaaagcccataattctgacactttggcgggtgatgaattacaggctttgcaatctg

SEQ ID NO: 103 - DNA, 370 bp, Artificial Sequence
  source 1..370: /mol_type="DNA" /note="subject" /organism="Artificial Sequence"
cgtgacaaggtgcaaattcttggttcgctggagttgcccaacggtgagatcaaacatgagcttgttgacttaacggttgaagatgctcgcatctttgagccattcaaacacaaggtaattagcatttcatgcggtgctatggctatcggtcgaaatgttgttttttatgttcgaaaaggtgcaaagcctgttttagcagatgtaatgtaattcatgaaaaaaaacagtgagttaggcttgccgactcgctgttttttcttttacttgatactattaactaaagtggggacaaaattgactaaaaaagacaataaaaaagcccataattctgatgctttggcgggcgacgaattacaggctttgcaatctg

SEQ ID NO: 104 - DNA, 52 bp, Artificial Sequence
  source 1..52: /mol_type="DNA" /note="query" /organism="Artificial Sequence"
ctaaggcagatcaacacagggatagaataacacgttttgggattttgaaaca

SEQ ID NO: 105 - RNA, 52 nt, Artificial Sequence
  source 1..52: /mol_type="RNA" /note="subject" /organism="Artificial Sequence"
cuaaugcagaucaacacagggauagaauaucacguuuuggacuuuugaaaca

SEQ ID NO: 106 - DNA, 112 bp, Artificial Sequence
  source 1..112: /mol_type="DNA" /note="query" /organism="Artificial Sequence"
aaggcagatcaacacagggatagaataacacgttttgggattttgaaacatagagcgaagctacaagaacaatatttgtggacgcaggttgatttcaaatctgaaggcgaag

SEQ ID NO: 107 - DNA, 119 bp, Artificial Sequence
  source 1..119: /mol_type="DNA" /note="subject" /organism="Artificial Sequence"
aaggagatcaacatagggatagaataacacgttttggcattttgaaacatagatcgaagcaacaagaaaactatttattttcgttagctaagattaaagaaaattatcatgccgatgta

SEQ ID NO: 108 - protein, 338 aa, Artificial Sequence
  SOURCE 1..338: /mol_type="protein" /note="query" /organism="Artificial Sequence"
LTKKDNKKAHNSDTLAGDELQALQSAKADQHRDRITRFGILKHRAKLQEQYLWTQVDFKSEGEDDLSNKALKAATKLKGCGQFLIFRNYYTIDQVKLEKFHVCGQHLLCPMCAGIRAARSMKRYLDRIHELMRQNPRLKPVLITLTVKNGEDLEERYNHLTSSFRKLLSRYRDYKKKGWGFNQFCKIDGAFYTTEYTYNEKTKQWHPHIHIFALLNEWIDQEELSETWHDITLDSYIIDIRRVKKTKEHGYSKAVAEVCKYALKFGDLSVENTWDAFLTLKGKRLTGSFGSMHGVKIPDKATDDMPLEELPYLEMFYRFVFDKKSYYNLEITKDVTPQ

SEQ ID NO: 109 - protein, 342 aa, Artificial Sequence
  SOURCE 1..342: /mol_type="protein" /note="subject" /organism="Artificial Sequence"
MLKKDNKKAHISEALAGGEIQALQSANADQHRDRITRFATLKHRAKNQENYLFTLAKFKENYEKDVKNEESIKALKSAQKLNECGNYLLFKNFYTIGEVKLSKLRTCGQHLLCPFCAAIRASRAIQKYVERIDQVLQENRKLKPVLITLTVKNGSDLAERSEHLMKSFRTLLERRRDYEKKGRGFNEFCKVQGAMYSYENTFNEKTGEWHPHIHMFALVDQWIDQQEFSEYWHSLTGDSMVVDVRRARKEKGYGYSKAAAEVCKYALKFGDLSVEKTWEAFKVLKGKRLTGSFGLLWGVKIPDSMTDDMPSEDLPYLEMLYKFAYSKKSYYDLLITRHVEPQ

SEQ ID NO: 110 - protein, 355 aa, Artificial Sequence
  SOURCE 1..355: /mol_type="protein" /note="query" /organism="Artificial Sequence"
KKDNKKAHNSDTLAGDELQALQSAKADQHRDRITRFGILKHRAKLQEQYLWTQVDFKSEGEDDLSNKALKAATKLKGCGQFLIFRNYYTIDQVKLEKFHVCGQHLLCPMCAGIRAARSMKRYLDRIHELMRQNPRLKPVLITLTVKNGEDLEERYNHLTSSFRKLLSRYRDYKKKGWGFNQFCKIDGAFYTTEYTYNEKTKQWHPHIHIFALLNEWIDQEELSETWHDITLDSYIIDIRRVKKTKEHGYSKAVAEVCKYALKFGDLSVENTWDAFLTLKGKRLTGSFGSMHGVKIPDKATDDMPLEELPYLEMFYRFVFDKKSYYNLEITKDVTPQTNSRQSEEAAPTTDTTGEN

SEQ ID NO: 111 - protein, 360 aa, Artificial Sequence
  SOURCE 1..360: /mol_type="protein" /note="subject" /organism="Artificial Sequence"
QKDIKKPLLSSTLVGGDNKGSNSVEADQHRDRITRFGILKHRSKQQENYLWTLAKYKENYQNDQPNEESVRATKSAQKLLGCGNFLLFKNFYTIDQVKLSKFHVCNQHLLCPFCAGIRASKAIQKYTERVDEVLSKKRTLKPVLITFTVKNGTDLGERSSHLMKSFRTLMERRRDYLKKGRGFNEFCKINGAMYSYENTYNEQTKEWHPHLHMFALLDDWIDQEELSQYWHSITGDSMIVDIRKVKKEKGLGYSKAAAEVCKYALKFGDLSVENTWEAFKILKGKRLSGAFGSLYGVKIPENLADEMPDENDLPYLEMLYKFVFGKKSYYDLTMTRHVEPRAQDDRPMEKELRRPTEGES

SEQ ID NO: 112 - protein, 232 aa, Artificial Sequence
  SOURCE 1..232: /mol_type="protein" /note="query" /organism="Artificial Sequence"
LQEQYLWTQVDFKSEGEDDLSNKALKAATKLKGCGQFLIFRNYYTIDQVKLEKFHVCGQHLLCPMCAGIRAARSMKRYLDRIHELMRQNPRLKPVLITLTVKNGEDLEERYNHLTSSFRKLLSRYRDYKKKGWGFNQFCKIDGAFYTTEYTYNEKTKQWHPHIHIFALLNEWIDQEELSETWHDITLDSYIIDIRRVKKTKEHGYSKAVAEVCKYALKFGDLSVENTWDAFL

SEQ ID NO: 113 - protein, 230 aa, Artificial Sequence
  SOURCE 1..230: /mol_type="protein" /note="subject" /organism="Artificial Sequence"
MQEQYLWTQVDFKVGSETSIKALKAATKLKGCGQFLLFRNYYTIDQIKLEKFHVCGQHLLCPMCAGIRAARSMNRYIQRIEEIMRQNRKLKPVLITLTVKNGEDLQERFEHLTGSFKTLLQRYRDFKKKGRGFNQFCKIDGGFYTTEYTYNETTQQWHPHIHIFALVTDRIDQEELAETWHDITLDSYIVDIRRVKKTKEHGYAKAVAEVCKYALKFSDLSTEKTFQAFF

SEQ ID NO: 114 - protein, 245 aa, Artificial Sequence
  SOURCE 1..245: /mol_type="protein" /note="query" /organism="Artificial Sequence"
MCAGIRAARSMKRYLDRIHELMRQNPRLKPVLITLTVKNGEDLEERYNHLTSSFRKLLSRYRDYKKKGWGFNQFCKIDGAFYTTEYTYNEKTKQWHPHIHIFALLNEWIDQEELSETWHDITLDSYIIDIRRVKKTKEHGYSKAVAEVCKYALKFGDLSVENTWDAFLTLKGKRLTGSFGSMHGVKIPDKATDDMPLEELPYLEMFYRFVFDKKSYYNLEITKDVTPQTNSRQSEEAAPTTDTTG

SEQ ID NO: 115 - protein, 247 aa, Artificial Sequence
  SOURCE 1..247: /mol_type="protein" /note="subject" /organism="Artificial Sequence"
FCAGIRASKSIQKYTDRVDEVLSKNRKLKPVLITFTVKNGTDLGERSSHLIKSFRTLLERRRDYLKKGRGFNEFCKIDGAMYSYENTFNESTKEWHPHLHLFALLDEWIDQEQLSELWHDITGDSYIVDVRKVKKSKDTGYAKAAAEVCKYALKFGDLTVENTWEAFKILKGKRLSGAFGSLYGVKIPDNPADDIDDSDLPYLEMVYKFVFGKKSYYDLTMTRHVEPQGQDNDDNEEKEGATSDRGG

SEQ ID NO: 116 - protein, 245 aa, Artificial Sequence
  SOURCE 1..245: /mol_type="protein" /note="query" /organism="Artificial Sequence"
CAGIRAARSMKRYLDRIHELMRQNPRLKPVLITLTVKNGEDLEERYNHLTSSFRKLLSRYRDYKKKGWGFNQFCKIDGAFYTTEYTYNEKTKQWHPHIHIFALLNEWIDQEELSETWHDITLDSYIIDIRRVKKTKEHGYSKAVAEVCKYALKFGDLSVENTWDAFLTLKGKRLTGSFGSMHGVKIPDKATDDMPLEELPYLEMFYRFVFDKKSYYNLEITKDVTPQTNSRQSEEAAPTTDTTGE

SEQ ID NO: 117 - protein, 245 aa, Artificial Sequence
  SOURCE 1..245: /mol_type="protein" /note="subject" /organism="Artificial Sequence"
CAAIRASRAIQKYVERIDQVLQENRKLKPVLITLTVKNGSDLAERSEHLMKSFRKLLDRRRDYEKKGRGFNEFCKVQGAMYSYENTFNEKTGEWHPHIHMFALVDQWIDQQEFSEYWHSLTGDSMVVDVRRAKKEKGHGYSKAAAEVCKYALKFGDLSVEKTWEAFKVLKGKRLTGSFGLLWGVKIPDTMTDDMPEEDLPYLEMLYKFAYGKKSYYDLLITRHVEPKAKDDNDEKEEPRQRRGGE

SEQ ID NO: 118 - protein, 228 aa, Artificial Sequence
  SOURCE 1..228: /mol_type="protein" /note="query" /organism="Artificial Sequence"
MCAGIRAARSMKRYLDRIHELMRQNPRLKPVLITLTVKNGEDLEERYNHLTSSFRKLLSRYRDYKKKGWGFNQFCKIDGAFYTTEYTYNEKTKQWHPHIHIFALLNEWIDQEELSETWHDITLDSYIIDIRRVKKTKEHGYSKAVAEVCKYALKFGDLSVENTWDAFLTLKGKRLTGSFGSMHGVKIPDKATDDMPLEELPYLEMFYRFVFDKKSYYNLEITKDVTPQ

SEQ ID NO: 119 - protein, 228 aa, Artificial Sequence
  SOURCE 1..228: /mol_type="protein" /note="subject" /organism="Artificial Sequence"
FCAAIRASRAIQKYVERIDQVLQENRKLKPVLITLTVKNGSDLAERSEHLMKSFRTLLERRRDYEKKGRGFNEFCKVQGAMYSYENTFNEKTGEWHPHIHMFALVDQWIDQQEFSEYWHSLTGDSMVVDVRRARKEKGYGYSKAAAEVCKYALKFGDLSVEKTWEAFKVLKGKRLTGSFGLLWGVKIPDSMTDDMPSEDLPYLEMLYKFAYSKKSYYDLLITRHVEPQ

SEQ ID NO: 120 - protein, 168 aa, Artificial Sequence
  SOURCE 1..168: /mol_type="protein" /note="query" /organism="Artificial Sequence"
MCAGIRAARSMKRYLDRIHELMRQNPRLKPVLITLTVKNGEDLEERYNHLTSSFRKLLSRYRDYKKKGWGFNQFCKIDGAFYTTEYTYNEKTKQWHPHIHIFALLNEWIDQEELSETWHDITLDSYIIDIRRVKKTKEHGYSKAVAEVCKYALKFGDLSVENTWDAFL

SEQ ID NO: 121 - protein, 168 aa, Artificial Sequence
  SOURCE 1..168: /mol_type="protein" /note="subject" /organism="Artificial Sequence"
MCAGIRAARSMNRYIQRIEEIMRQNRKLKPVLITLTVKNGEDLQERFEHLTGSFKTLLQRYRDFKKKGRGFNQFCKIDGGFYTTEYTYNETTQQWHPHIHIFALVTDRIDQEELAETWHDITLDSYIVDIRRVKKTKEHGYAKAVAEVCKYALKFSDLSTEKTFQAFF

SEQ ID NO: 122 - protein, 78 aa, Artificial Sequence
  SOURCE 1..78: /mol_type="protein" /note="query" /organism="Artificial Sequence"
SDEDLKPITIRLADSEIQAYDTVAKSMGLTRQDFLSHVIRSNFRQALKEFVVGYTSSNPSTPLSVLFNSNTDNDEVKL

SEQ ID NO: 123 - protein, 70 aa, Artificial Sequence
  SOURCE 1..70: /mol_type="protein" /note="subject" /organism="Artificial Sequence"
ADGLIRPPSQREIQAHSTAKYGALARQRYRMETSFPPWLKSLTVGSAVSTPCTPLKHLQNCNRNTSKLKL

SEQ ID NO: 124 - protein, 60 aa, Artificial Sequence
  SOURCE 1..60: /mol_type="protein" /note="subject" /organism="Artificial Sequence"
FLFRSIAVLITTNNWDMTEIFLFALSVLLLISCIVYYYTVPDKEMILNRRDGLVSFPAFT

SEQ ID NO: 125 - protein, 79 aa, Artificial Sequence
  SOURCE 1..79: /mol_type="protein" /note="query" /organism="Artificial Sequence"
MLFKSLGVAIATNNASNSDEDLKPITIRLADSEIQAYDTVAKSMGLTRQDFLSHVIRSNFRQALKEFVVGYTSSNPSTP

SEQ ID NO: 126 - DNA, 19 bp, Artificial Sequence
  source 1..19: /mol_type="DNA" /note="Nn forward primer" /organism="Artificial Sequence"
ggattaatgccaatgatcc

SEQ ID NO: 127 - DNA, 18 bp, Artificial Sequence
  source 1..18: /mol_type="DNA" /note="Xn reverse primer" /organism="Artificial Sequence"
ctttgcctgtttctctcg

SEQ ID NO: 128 - DNA, 24 bp, Artificial Sequence
  source 1..24: /mol_type="DNA" /note="No forward primer" /organism="Artificial Sequence"
gaggacgaattaatattacaagtc

SEQ ID NO: 129 - DNA, 19 bp, Artificial Sequence
  source 1..19: /mol_type="DNA" /note="Xo reverse primer" /organism="Artificial Sequence"
gttctcgttttcttggtaa

SEQ ID NO: 130 - DNA, 24 bp, Artificial Sequence
  source 1..24: /mol_type="DNA" /note="Nd forward primer" /organism="Artificial Sequence"
cagattgcaaagcctgtaattcat

SEQ ID NO: 131 - DNA, 24 bp, Artificial Sequence
  source 1..24: /mol_type="DNA" /note="Xd reverse primer" /organism="Artificial Sequence"
ctaaggcagatcaacacagggata

SEQ ID NO: 132 - DNA, 19 bp, Artificial Sequence
  source 1..19: /mol_type="DNA" /note="forward primer" /organism="Artificial Sequence"
ggattaatgccaatgatcc

SEQ ID NO: 133 - DNA, 18 bp, Artificial Sequence
  source 1..18: /mol_type="DNA" /note="reverse primer" /organism="Artificial Sequence"
cgagagaaacaggcaaag

SEQ ID NO: 134 - DNA, 24 bp, Artificial Sequence
  source 1..24: /mol_type="DNA" /note="forward primer" /organism="Artificial Sequence"
gaggacgaattaatattacaagtc

SEQ ID NO: 135 - DNA, 20 bp, Artificial Sequence
  source 1..20: /mol_type="DNA" /note="reverse primer" /organism="Artificial Sequence"
ttaccaagaaaagcgagaac

SEQ ID NO: 136 - DNA, 24 bp, Artificial Sequence
  source 1..24: /mol_type="DNA" /note="forward primer" /organism="Artificial Sequence"
ctaatgcagatcaacacagggata

SEQ ID NO: 137 - DNA, 22 bp, Artificial Sequence
  source 1..22: /mol_type="DNA" /note="reverse primer" /organism="Artificial Sequence"
gaattacaggctttgcaatctg

SEQ ID NO: 138 - protein, 5 aa, Artificial Sequence
  SOURCE 1..5: /mol_type="protein" /note="motif" /organism="Artificial Sequence"
LLTYA

SEQ ID NO: 139 - protein, 7 aa, Artificial Sequence
  SOURCE 1..7: /mol_type="protein" /note="motif" /organism="Artificial Sequence"
HLHAFVD

SEQ ID NO: 140 - protein, 5 aa, Artificial Sequence
  SOURCE 1..5: /mol_type="protein" /note="motif" /organism="Artificial Sequence"
YAIKD

SEQ ID NO: 141 - protein, 5 aa, Artificial Sequence
  SOURCE 1..5: /mol_type="protein" /note="motif" /organism="Artificial Sequence"
VFDDI

SEQ ID NO: 142 - protein, 5 aa, Artificial Sequence
  SOURCE 1..5: /mol_type="protein" /note="motif" /organism="Artificial Sequence"
LLKMP

SEQ ID NO: 143 - protein, 7 aa, Artificial Sequence
  SOURCE 1..7: /mol_type="protein" /note="motif" /organism="Artificial Sequence"
HYHIYLG

SEQ ID NO: 144 - protein, 5 aa, Artificial Sequence
  SOURCE 1..5: /mol_type="protein" /note="motif" /organism="Artificial Sequence"
YVGKD

SEQ ID NO: 145 - protein, 5 aa, Artificial Sequence
  SOURCE 1..5: /mol_type="protein" /note="motif" /organism="Artificial Sequence"
VFDDI

SEQ ID NO: 146 - protein, 5 aa, Artificial Sequence
  SOURCE 1..5: /mol_type="protein" /note="motif" /organism="Artificial Sequence"
LLTYP

SEQ ID NO: 147 - protein, 7 aa, Artificial Sequence
  SOURCE 1..7: /mol_type="protein" /note="motif" /organism="Artificial Sequence"
HLHAFVD

SEQ ID NO: 148 - protein, 5 aa, Artificial Sequence
  SOURCE 1..5: /mol_type="protein" /note="motif" /organism="Artificial Sequence"
YAIKD

SEQ ID NO: 149 - protein, 5 aa, Artificial Sequence
  SOURCE 1..5: /mol_type="protein" /note="motif" /organism="Artificial Sequence"
IFDDF

SEQ ID NO: 150 - protein, 16 aa, Artificial Sequence
  SOURCE 1..16: /mol_type="protein" /note="motif" /organism="Artificial Sequence"
AVFDVGGFHPNISITK

SEQ ID NO: 151 - protein, 16 aa, Artificial Sequence
  SOURCE 1..16: /mol_type="protein" /note="motif" /organism="Artificial Sequence"
TAFDYFGAHGNIKSIR

SEQ ID NO: 152 - protein, 16 aa, Artificial Sequence
  SOURCE 1..16: /mol_type="protein" /note="motif" /organism="Artificial Sequence"
RAFDVEGCHPNVSPSR

SEQ ID NO: 153 - DNA, 23 bp, Artificial Sequence
  source 1..23: /mol_type="DNA" /note="forward primer" /organism="Artificial Sequence"
gacttctgattgattgatgcctg

SEQ ID NO: 154 - DNA, 24 bp, Artificial Sequence
  source 1..24: /mol_type="DNA" /note="reverse primer" /organism="Artificial Sequence"
cctgttgaataccgcttaaatact

SEQ ID NO: 155 - DNA, 2149 bp, Artificial Sequence
  source 1..2149: /mol_type="DNA" /note="HCBI8.215" /organism="Artificial Sequence"
taatgttatctacctttctgttgtgtcggtgtcactttacttggtatatataggcggttgtcccgcggagaaatttatttcgcaaagaggggtatgttgcatttacaaaatggcgttccggaatcggcgttttcaggcggggcgcaggcgtcgttttactccacggaggtccacttttcgccgacgatctttccgcaatggtcggtcacgtacgacaaggcggtattcacggccacgcacgaatgtgcgtcgtgtgcgcaatctcgcgtctcggaagtgtcgcgacaatatgatttgtactcctattgacgacacgggtactcctcagactcccggacccgtatctatggatgcatcatctgtttacgggttcatcttttcaccaactgcacggaccgcaggtactcaacttgagagcggtgagcgggtcaatgcacctagctcggcccagcggaggaagagcaaatgttacgttcggggttacggagaaactgtcgaaattcagacggatgacgcgtcgccatgggtatggcgtcgtattgtgttcagcactattggcttggcgtctcagtttgaccccggtcttttgtacaacaatgacgaaacccgtggctggggtcgcagcctgttcaatatccggagtggtacgcagcaggcatccattcttgagggcgttgtttttaggtacctattccagggtaccgagggtgtcgattgggccaatgtcatgactgctactacggcccctcggcatgtcagggtttattccgatcggcgccgtgttattcaatcccccaactcggaggggggtactattcgactatcgaagcattacgatggtattaatcggagcattatttacgacgatgtggaaattggagcgggagcgaaggctacgaatgccattgcgagtggaactccatatgggaatatgggagatttgtttgttcttgatttcttttcgagtgcatcggatgatgagaccagcggagcgtctttccagcctcatgggaagttttattggcatgaagggcaatctgcttagctatagaggggagtcgtgacttctacaaaaatacaattcttgtccatccagtcctgatccaccccttctgtgatgggatactcatttgatatccaaatacatggtttcccccacttaattgccttcttcttcttgtacttgtctgtagaatagaagtctagctggtttcccagccatgacttgtactgtgggaagaattgagtcctccggcgatgtcatcaaagacggcatacttgacatcctcaagggattcctccagtgagaagagccgccaaaataggcgtgcttggcgagagatcttgcccacatagtcttgccagttcttgagggtccatagaggaccagtgactttcccctgcctaacacattagccgttagggttagggttaccctttagggttagggttagggttagggttagggttagggttagggttagggttaccctttagggttagaggattatgaaaatgtcgtggtgtgtgtgtactaaccccttactgtggcatcccatccaatgtagtcctcagcccactgattgagctcaggaaactgcgaagtgtcgaattcatactctgggtcgtgtcgatatgggtctggatccacacgatagtgccagtcggcatatttctcgagtgacgggaagctggtgagtagaagtcttgggtccaaatcacggacagcttcgaaaaactccgctcgagtcggtgccaagacgatttgatggtgcttattctcaactccagcgcttgcatctgctgctggtcgttcgagtcctccagcgacaacatcccatccttgatcgcgtaatcataatggacttgagggtcgcgcttagtaattgagatgttagggtggaaacctccaacatcaaagacagcagcacgtcttgattgaaatcgtcgtccaaaatccacaaaagcgtgcagatgagttccgccatcagagtgggcttctcttccaatgatgcattctcctccaaggtcaccaatgtgtgaaacaatagtgaatgggtcgaggccgccgcattgagcgtaggtgagaagcgcatatcgggcatagaagcgaaatgtcgacattgagggtgacacagaaaggtaggtt

SEQ ID NO: 156 - DNA, 286 bp, Artificial Sequence
  source 1..286: /mol_type="DNA" /note="query" /organism="Artificial Sequence"
cctccagcgacaacatcaccatccttgatcgcgtaatcataatggacttgagggtcgcgcttagtaattgagatgttagggtggaaacctccaacatcaaagacagcagcacgtcttgattgaaatcgtcgtccaaaatccacaaaagcgtgcagatgagttccgccatcagagtgggcttctcttccaatgatgcattctcctccaaggtcaccaatgtgtgaaacaatagtgaatgggtcgaggccgccgcattgagcgtaggtgagaagcgcatatcgggcat

SEQ ID NO: 157 - DNA, 286 bp, Artificial Sequence
  source 1..286: /mol_type="DNA" /note="subject" /organism="Artificial Sequence"
cctccagcgaccacgtctccatctttgatcgcatagtcgtaaccgccttccggctttccgtaagatggaacaaggttcgggtggcggcctccaacatcaaagacatcggatcgtcgggatcgaaatcggcgggagaaatcacagaaagcatggagatgagtacctccatcagcgtgcaactctcgtccaatgatacactcagctccaaggaacgccaaatggtcattaacggtccatgcatcaagagtgccgcactgtgcgtacgtgagaagaaagtatcggccat

SEQ ID NO: 158 - DNA, 300 bp, Artificial Sequence
  source 1..300: /mol_type="DNA" /note="query" /organism="Artificial Sequence"
agtcctccagcgacaacatcaccatccttgatcgcgtaatcataatggacttgagggtcgcgcttagtaattgagatgttagggtggaaacctccaacatcaaagacagcagcacgtcttgattgaaatcgtcgtccaaaatccacaaaagcgtgcagatgagttccgccatcagagtgggcttctcttccaatgatgcattctcctccaaggtcaccaatgtgtgaaacaatagtgaatgggtcgaggccgccgcattgagcgtaggtgagaagcgcatatcgggcatagaagcgaaat

SEQ ID NO: 159 - DNA, 300 bp, Artificial Sequence
  source 1..300: /mol_type="DNA" /note="query" /organism="Artificial Sequence"
agccctccagcgaccacgtctccatctttgatcgcatagtcataaccgccttccggccttcctcgagatgcttcaatgttagggtggaagcctccaacatcaaacacatcgggtcttcgggatcgaaactttcgggagaaatcgcagaaagcatggagatgagtacccccatcagcgtgatgctctcgtccaatgatacactcaccgccaaggaatgccagatggtcattaacggcccatgcatcaaggtcgccgcactgtgcgtaggtaaggaggacatagcgtgcttggaattgaaat

SEQ ID NO: 160 - DNA, 282 bp, Artificial Sequence
  source 1..282: /mol_type="DNA" /note="query" /organism="Artificial Sequence"
cctccagcgacaacatcaccatccttgatcgcgtaatcataatggacttgagggtcgcgcttagtaattgagatgttagggtggaaacctccaacatcaaagacagcagcacgtcttgattgaaatcgtcgtccaaaatccacaaaagcgtgcagatgagttccgccatcagagtgggcttctcttccaatgatgcattctcctccaaggtcaccaatgtgtgaaacaatagtgaatgggtcgaggccgccgcattgagcgtaggtgagaagcgcatatcgg

SEQ ID NO: 161 - DNA, 282 bp, Artificial Sequence
  source 1..282: /mol_type="DNA" /note="subject" /organism="Artificial Sequence"
cctccagcgaccacgtctccatctttgatcgcatagtcataaccgccttccgggcttccgtaagatggaacaaggttcggatggcggcctccaacatcaaagacatcggatcttctggatcgaaacttccgggagaaatcgacgaaagcatggagatgagtacctccatcagcatgcaattctcgtccaatgatacactcaccgccaagaaatgccatatggtcattaacggcccatgcatcaaggtcgccgcactgtgcgtaggtaaggagggcataacgg

SEQ ID NO: 162 - protein, 287 aa, Artificial Sequence
  SOURCE 1..287: /mol_type="protein" /note="query" /organism="Artificial Sequence"
STFRRRSFRNGRSRTTRRYSRPRTNVRRVRNLASRKCRDNMICTPIDDTGTPQTPGPVSMDASSVYGFIFSPTARTAGTQLESGERVNAPSSAQRRKSKCYVRGYGETVEIQTDDASPWVWRRIVFSTIGLASQFDPGLLYNNDETRGWGRSLFNIRSGTQQASILEGVVFRYLFQGTEGVDWANVMTATTAPRHVRVYSDRRRVIQSPNSEGGTIRLSKHYDGINRSIIYDDVEIGAGAKATNAIASGTPYGNMGDLFVLDFFSSASDDETSGASFQPHGKFYWHE

SEQ ID NO: 163 - protein, 273 aa, Artificial Sequence
  SOURCE 1..273: /mol_type="protein" /note="subject" /organism="Artificial Sequence"
SSKKRRSYVGRRLSSRRTTKTVMKRTSRRRILNISSQKKRNNAQPVNFNYLGESPIPGSKVMGSDRTTYLLWRPTALTDDTDIYSSASRGAQQIYWRGIKERAEVGTSSGAAWRWRRIVFEAKSLNINGLISNVETSAGFNRAMVELSGDPPANLRNSLESFLFQGSVGVDWNTVFNAKVDNNRCRLLSDKVRHLQSGNDRGRFYTFRQWIPLNKTMVYNDDEVGDDKQSNTFASPGRKGMGDVYVYDMFQCLTSDAINTLNFNPQATLYWHE

SEQ ID NO: 164 - protein, 283 aa, Artificial Sequence
  SOURCE 1..283: /mol_type="protein" /note="query" /organism="Artificial Sequence"
RRRSFRNGRSRTTRRYSRPRTNVRRVRNLASRKCRDNMICTPIDDTGTPQTPGPVSMDASSVYGFIFSPTARTAGTQLESGERVNAPSAQRRKSKCYVRGYGETVEIQTDDASPWVWRRIVFSTIGLASQFDPGLLYNNDETRGWGRSLFNIRSGTQQASILEGVVFRYLFQGTEGVDWANVMTATTAPRHVRVYSDRRRVIQSPNSEGGTIRLSKHYDGINRSIIYDDVEIGAGAKATNAIASGTPYGNMGDLFVLDFFSSASDDETSGASFQPHGKFYWHE

SEQ ID NO: 165 - protein, 277 aa, Artificial Sequence
  SOURCE 1..277: /mol_type="protein" /note="subject" /organism="Artificial Sequence"
RRRSYPTTRRRYPRKTLAKRILNISSTKKRDNMMSYTNVTVANPINGQTYAAGPAVLRGDQTYIFAWIPTARDLIRADGEPNTPVWLAGRTRQTCYMRGLKEAMNVRTNSGSSWQWRRICFTMKGPNLIGYATTGSNLWQETSNGMVRTMNNVNTKPLGNEILAQLFRGAQNQDWLNVFNAQTDTTKFTIKYDRTISIASGNEQGLVRTYKHWYPMNKNLVYNDDENADGVLTSYTSTNGKPGMGDYYVVDFFQPADGADASDTLALLPEATLYWHE

SEQ ID NO: 166 - protein, 261 aa, Artificial Sequence
  SOURCE 1..261: /mol_type="protein" /note="query" /organism="Artificial Sequence"
RRVRNLASRKCRDNMICTPIDDTGTPQTPGPVSMDASSVYGFIFSPTARTAGTQLESGERVNAPSSAQRRKSKCYVRGYGETVEIQTDDASPWVWRRIVFSTIGLASQFDPGLLYNNDETRGWGRSLFNIRSGTQQASILEGVVFRYLFQGTEGVDWANVMTATTAPRHVRVYSDRRRVIQSPNSEGGTIRLSKHYDGINRSIIYDDVEIGAGAKATNAIASGTPYGNMGDLFVLDFFSSASDDETSGASFQPHGKFYWHE

SEQ ID NO: 167 - protein, 246 aa, Artificial Sequence
  SOURCE 1..246: /mol_type="protein" /note="subject" /organism="Artificial Sequence"
RRILNVSSKKKRDNMINVSFSPTGINPAVRGFIATGAAPTMLVWCATARDRVSNASNPTADSVRESQTCYMRGLKEHIRINTNNPTSWLWRRICFTAKGLFSGLGTSADSVETSNGWVRALMDQTGTSFGTSLTNLLFAGTNGVDWNDTFTANTDSTNVKIMYDKTFTINSGVSGVIRDYKMWHGMNKNIVYGEDENGEGEINNRYSTIGRPGMGDYYVVDLLASNSSAAADTLTFSTEATLYWHE

SEQ ID NO: 168 - protein, 287 aa, Artificial Sequence; identical to SEQ ID NO: 162
  SOURCE 1..287: /mol_type="protein" /note="query" /organism="Artificial Sequence"

SEQ ID NO: 169 - protein, 273 aa, Artificial Sequence; identical to SEQ ID NO: 163
  SOURCE 1..273: /mol_type="protein" /note="subject" /organism="Artificial Sequence"

SEQ ID NO: 170 - protein, 284 aa, Artificial Sequence
  SOURCE 1..284: /mol_type="protein" /note="query" /organism="Artificial Sequence"
RRRSFRNGRSRTTRRYSRPRTNVRRVRNLASRKCRDNMICTPIDDTGTPQTPGPVSMDASSVYGFIFSPTARTAGTQLESGERVNAPSSAQRRKSKCYVRGYGETVEIQTDDASPWVWRRIVFSTIGLASQFDPGLLYNNDETRGWGRSLFNIRSGTQQASILEGVVFRYLFQGTEGVDWANVMTATTAPRHVRVYSDRRRVIQSPNSEGGTIRLSKHYDGINRSIIYDDVEIGAGAKATNAIASGTPYGNMGDLFVLDFFSSASDDETSGASFQPHGKFYWHE

SEQ ID NO: 171 - protein, 277 aa, Artificial Sequence; identical to SEQ ID NO: 165
  SOURCE 1..277: /mol_type="protein" /note="subject" /organism="Artificial Sequence"

SEQ ID NO: 172 - protein, 261 aa, Artificial Sequence; identical to SEQ ID NO: 166
  SOURCE 1..261: /mol_type="protein" /note="query" /organism="Artificial Sequence"

SEQ ID NO: 173 - protein, 246 aa, Artificial Sequence; identical to SEQ ID NO: 167
  SOURCE 1..246: /mol_type="protein" /note="subject" /organism="Artificial Sequence"

SEQ ID NO: 174 - protein, 186 aa, Artificial Sequence
  SOURCE 1..186: /mol_type="protein" /note="query" /organism="Artificial Sequence"
FRFYARYALLTYAQCGGLDPFTIVSHIGDLGGECIIGREAHSDGGTHLHAFVDFGRRFQSRRAAVFDVGGFHPNISITKRDPQVHYDYAIKDGDVVAGGLERPAADASAGVENKHHQIVLAPTRAEFFEAVRDLDPRLLLTSFPSLEKYADWHYRVDPDPYRHDPEYEFDTSQFPELNQWAEDYIG

SEQ ID NO: 175 - protein, 186 aa, Artificial Sequence
  SOURCE 1..186: /mol_type="protein" /note="subject" /organism="Artificial Sequence"
FQFQARYVLLTYAQCGDLDAWAVNDHLAFLGGECIIGREHHADGGTHLHAFCDFSRKFRSRRPDVFDVGGFHPNIEASRGRPEGGYDYAIKDGDVVAGGLSRPGGRGVYEDVSSWSIIVSQESEGDFWECVARLDPRSLCTNYNSLRAYANWKYRPTPVQYVHPAGVEFELGMVPELAVWREIALG

SEQ ID NO: 176 - protein, 188 aa, Artificial Sequence
  SOURCE 1..188: /mol_type="protein" /note="query" /organism="Artificial Sequence"
MSTFRFYARYALLTYAQCGGLDPFTIVSHIGDLGGECIIGREAHSDGGTHLHAFVDFGRRFQSRRAAVFDVGGFHPNISITKRDPQVHYDYAIKDGDVVAGGLERPAADASAGVENKHHQIVLAPTRAEFFEAVRDLDPRLLLTSFPSLEKYADWHYRVDPDPYRHDPEYEFDTSQFPELNQWAEDYI

SEQ ID NO: 177 - protein, 191 aa, Artificial Sequence
  SOURCE 1..191: /mol_type="protein" /note="subject" /organism="Artificial Sequence"
MSSFRFQARYALLTYAQCGDLDPFAVSDHLSGLRAECIIGRETHADEGIHLHAFVDFGVKFSTRNVRVFDVQGHHPNVEPSRGRPAGGYDYAIKDGDVVAGGLDRPADDGGVGVSKTTQKWATIVGAQTRDEFWALLAELDPGAMVRSFTQCRAYADHRFRESPERYVTPESIIIDTGHVDGLNEWALSNI

SEQ ID NO: 178 - protein, 183 aa, Artificial Sequence
  SOURCE 1..183: /mol_type="protein" /note="query" /organism="Artificial Sequence"
RYALLTYAQCGGLDPFTIVSHIGDLGGECIIGREAHSDGGTHLHAFVDFGRRFQSRRAAVFDVGGFHPNISITKRDPQVHYDYAIKDGDVVAGGLERPAADASAGVENKHHQIVLAPTRAEFFEAVRDLDPRLLLTSFPSLEKYADWHYRVDPDPYRHDPEYEFDTSQFPELNQWAEDYIGWD

SEQ ID NO: 179 - protein, 183 aa, Artificial Sequence
  SOURCE 1..183: /mol_type="protein" /note="subject" /organism="Artificial Sequence"
RYALLTYAQCGDLDAWAVNDHMAFLGGECIIGRELHADGGTHLHAFVDFSRKFRSRRSDVFDVGGRHPNLVPSYGSPEGGYDYAIKDGDVVAGGLSRPSGRGVYEDVSSWSIIVSQESEGDFWECVARLDPRSLCTNYNSLRAYANWKYQPLPVRYEHPAGVKFELGMVPELAVWREVALGVD

SEQ ID NO: 180 - protein, 102 aa, Artificial Sequence
  SOURCE 1..102: /mol_type="protein" /note="query" /organism="Artificial Sequence"
MWARSLAKHAYFGGLFSLEESLEDVKYAVFDDIAGGLKFFPQYKSWLGNQLDFYSTDKYKKKKAIKWGKPCIWISNEYPITEGVDQDWMDKNCIFVEVTTPL

SEQ ID NO: 181 - protein, 103 aa, Artificial Sequence
  SOURCE 1..103: /mol_type="protein" /note="subject" /organism="Artificial Sequence"
LWARSLGNHAYFGGLFSLEEELEGVDYAIFDDMQGGLKFFHSYKFWLGAQSQFWATDKYRGKKLIHWGRPSIYICNQNPLCDEGVDHDWLIGNCDFVEITESL

SEQ ID NO: 182 - protein, 103 aa, Artificial Sequence
  SOURCE 1..103: /mol_type="protein" /note="query" /organism="Artificial Sequence"
MWARSLAKHAYFGGLFSLEESLEDVKYAVFDDIAGGLKFFPQYKSWLGNQLDFYSTDKYKKKKAIKWGKPCIWISNEYPITEGVDQDWMDKNCIFVEVTTPLY

SEQ ID NO: 183 - protein, 104 aa, Artificial Sequence
  SOURCE 1..104: /mol_type="protein" /note="subject" /organism="Artificial Sequence"
LWARSLGRHAYFGGLFCLDESLEDVDYAVFDDMQGGLEFFHAYKFWLGAQKQFYATDKYRGKQLVNWGRPSIYISNTNPLADKGADVDWLMGNCVIVHVDRPIF

SEQ ID NO: 184 - protein, 102 aa, Artificial Sequence; identical to SEQ ID NO: 180
  SOURCE 1..102: /mol_type="protein" /note="query" /organism="Artificial Sequence"

SEQ ID NO: 185 - protein, 105 aa, Artificial Sequence
  SOURCE 1..105: /mol_type="protein" /note="subject" /organism="Artificial Sequence"
VWARSLGDHAYFGGLFSMDEDISSATYAVFDDFGGLKFLPSYKFWMGHQKQFYVTDKYKGKKLVEWGRPSIWINNEDPREEHGVRCDEIEWLEQNCIFIRLDSTI

SEQ ID NO: 186 - DNA, 2120 bp, Artificial Sequence
  source 1..2120: /mol_type="DNA" /note="HCBI9.212" /organism="Artificial Sequence"
atttttcgaccagtaaaaaatggcttacggattccgccgccgctttggtcgctcccgtcgctcgtaccgacgaaggcccgttcgccgctattcccgaaggggtagaagcgggtatggtcgtggcggttacaaccgtcggcgttatcgtcgtcgtcgccgctcttggattagtccttacaacaaaaagcatgacgtgattaagggggcgcatgattcgaatgataattcgttcgcccctataggtgcccccaacaccttttttgggttctgcccaacctacatgcccaacgccgttgctggggatactggtcacaatcctcaaaaggttcggaccagtaagaatgttgggttcagtggatatcaggaacgtgttcatattgctacggctgaatctttgatttggcgtcgcatggttatttggtcatataaccggcttgagaatacggccggtccgacgaagacggatgatcagggtacttcgtacacgacacgtcagcttaccccgctccaattaaacgaaggggtccgtgcgtttttgttccgaggtactcagggtatcgattacactgagaacaccttgcatgaggctccgctgaattccgatcactttaccgttgcgtatgatcgtacacgtgtgttacagcctcgtcgtcctactggtgacgaatacggtcatatttttaatatgaagttctggaaccctggtggaaggattatttactcggatgatgaggatggtttacagaagggtcctcttgtgaacggatggtcttctcttggacgtgtgtctaagggaaacatgtatatttttgatgtcttttctacggggtattctttgagtagtaatactccttctattgctagatttgctccgactgggactcgttactggacggagggttagatacaatacaaattggatccaccacattgattatgtgacagttgttcataagccaatcgtagtccacccctttagcgaagtgtgggtcctcgttcatgcacatgattgagggtttgccccagtagatcgttcgcttctttcggtacttgtccgtgatgacgaattgtttttgtgcgcctagccaccccttgtatgagtggaagtattcgaatcctccctggatgtcgtcgaagacggcgtattgacaatcgtcggagaattcgtccatgttgaattgtaggttgaagtacgcatggtgtcccaacgatctggcgtatagcgtctttccggttcttgttggtccccataaaatgagtgatttaactctgcccaagtaaagatcagtaatggggttcggggcgaagccctgaagcggacaagatttgatcgtgcgaggacgctacgtcggccgcagcgccagcagacttacctctcgggtctacagtccccaatggctgcctgattctcccactcggagatctcaggatagcgttctctctccacaatgatgggcggcgcctcgtattccggtttctcgtcggggtaataaaaattggcgtattcgatgatgcgctgattggtagcaaccaatctcttggagcttgttgacggacagccgacagaaatgattctttagtgtcgcagctgatgatatcagcccacttatttgaattatccccgtcacatgagcgagcatctgctgggggctcgccgtgctcaagtcggatgtctccatccttgccgacataatcgaagaccttgtgtggagttcgacgaatcgatttaatattgccgtgagctccaaagtagtcgaacgcagttgccgagttgacagtgacaatcttgtcgaagccaagatatatgtggtaatgaattcctccatccgaatggcgctctcgtccgagtcgacagcataaaggatttccaaaattcgctgtgacacgttcaaggaaaggagttcctgcgtcgaattcatgttggaggtgttcggggacttgtggaaacgtaatgataagatttcttgctctgacttggaatcgtcgaggcattttaaggagtcgttcacgtgacgtgtgcaaatagagagagacttggctaatattatctctctctatttgcagtttgcacattgcacatggctgcctataaatacccctcatcccccctgcggtgagtc

SEQ ID NO: 187 - DNA, 146 bp, Artificial Sequence
  source 1..146: /mol_type="DNA" /note="query" /organism="Artificial Sequence"
gggtcctcgttcatgcacatgattgagggtttgccccagtagatcgttcgcttctttcggtacttgtccgtgatgacgaattgtttttgtgcgcctagccaccccttgtatgagtggaagtattcgaatcctccctggatgtcgtc

SEQ ID NO: 188 - DNA, 146 bp, Artificial Sequence
  source 1..146: /mol_type="DNA" /note="subject" /organism="Artificial Sequence"
gggtcctcgttcataagccagatagtggggcgcccccactggatggttgtcttccctcggtayttgtcggtgacggtgaatgtttgttgtgcaccyagccacccyttgtaggaaggaaagaattggaagtttccttgcatatcgtc

SEQ ID NO: 189 - DNA, 71 bp, Artificial Sequence
  source 1..71: /mol_type="DNA" /note="query" /organism="Artificial Sequence"
tgtgcgcctagccaccccttgtatgagtggaagtattcgaatcctccctggatgtcgtcgaagacggcgta

SEQ ID NO: 190 - DNA, 71 bp, Artificial Sequence
  source 1..71: /mol_type="DNA" /note="subject" /organism="Artificial Sequence"
tgagcaccgagccactccttgtatccgtgaaagaatccaaaaccacctctgatgtcgtcgaagacggcgta

SEQ ID NO: 191 - DNA, 102 bp, Artificial Sequence
  source 1..102: /mol_type="DNA" /note="query" /organism="Artificial Sequence"
tcggtacttgtccgtgatgacgaattgtttttgtgcgcctagccaccccttgtatgagtggaagtattcgaatcctccctggatgtcgtcgaagacggcgta

SEQ ID NO: 192 - DNA, 102 bp, Artificial Sequence
  source 1..102: /mol_type="DNA" /note="subject" /organism="Artificial Sequence"
tctgtacttgtccgtaactgtaaacttggactgcgcccccaaccaccccttgtatgacgggaaatacttgaatccgccctgcatatcatcaaatactgcata

SEQ ID NO: 193 - protein, 276 aa, Artificial Sequence
  SOURCE 1..276: /mol_type="protein" /note="query" /organism="Artificial Sequence"
RRPVRRYSRRGRSGYGRGGYNRRRYRRRRRSWISPYNKKHDVIKGAHDSNDNSFAPIGAPNTFFGFCPTYMPNAVAGDTGHNPQKVRTSKNVGFSGYQERVHIATAESLIWRRMVIWSYNRLENTAGPTKTDDQGTSYTTRQLTPLQLNEGVRAFLFRGTQGIDYTENTLHEAPLNSDHFTVAYDRTRVLQPRRPTGDEYGHIFNMKFWNPGGRIIYSDDEDGLQKGPLVNGWSSLGRVSKGNMYIFDVFSTGYSLSSNTPSIARFAPTGTRYWTE

SEQ ID NO: 194 - protein, 287 aa, Artificial Sequence
  SOURCE 1..287: /mol_type="protein" /note="subject" /organism="Artificial Sequence"
RRKYTRTIRRGRAGSSKKRRSYVGRRLSSRRTTKTVMKRTSRRRILNISSQKKRNNAQPVNFNYLGESPIPGSKVMGSDRTTYLLWRPTALTDDTDIYSSASRGAQQIYWRGIKERAEVGTSSGAAWRWRRIVFEAKSLNINGLISNVETSAGFNRAMVELSGDPPANLRNSLESFLFQGSVGVDWNTVFNAKVDNNRCRLLSDKVRHLQSGNDRGRFYTFRQWIPLNKTMVYNDDEVGDDKQSNTFASPGRKGMGDVYVYDMFQCLTSDAINTLNFNPQATLYWHE

SEQ ID NO: 195 - protein, 293 aa, Artificial Sequence
  SOURCE 1..293: /mol_type="protein" /note="query" /organism="Artificial Sequence"
MAYGFRRRFGRSRRSYRRRPVRRYSRRGRSGYGRGGYNRRRYRRRRRSWISPYNKKHDVIKGAHDSNDNSFAPIGAPNTFFGFCPTYMPNAVAGDTGHNPQKVRTSKNVGFSGYQERVHIATAESLIWRRMVIWSYNRLENTAGPTKTDDQGTSYTTRQLTPLQLNEGVRAFLFRGTQGIDYTENTLHEAPLNSDHFTVAYDRTRVLQPRRPTGDEYGHIFNMKFWNPGGRIIYSDDEDGLQKGPLVNGWSSLGRVSKGNMYIFDVFSTGYSLSSNTPSIARFAPTGTRYWTE

SEQ ID NO: 196 - protein, 302 aa, Artificial Sequence
  SOURCE 1..302: /mol_type="protein" /note="subject" /organism="Artificial Sequence"
SMAYARRRFTSSRARKPIRRSRRPAGKRRSYRRSTRKRGMSTRTLLNKTSQKKRDNMLSFSNTTAEDPFSTDYTIGPAVMRRPVGADLPAEFIYVWNATGRPHELSTGFRGSKIDTSLRTNTTIFAVGLKERIKLETNNSAPWRWRRICFTSKNDYGEADPDESDYFRRTSNGMVRLLRAQSQAEEINDDVFDGQRNVDWLSAITAPINRRHVSVHYDRTRTIQSGNQSGVTRTYRQWHPMRKNVVYADEQAGEGMVDSGVSVTGKVGMGNYYVMDIFTKHGLNDDQSTLSYEPESTFFWHE

SEQ ID NO: 197 - protein, 283 aa, Artificial Sequence
  SOURCE 1..283: /mol_type="protein" /note="query" /organism="Artificial Sequence"
RSRRSYRRRPVRRYSRRGRSGYGRGGYNRRRYRRRRRSWISPYNKKHDVIKGAHDSNDNSFAPIGAPNTFFGFCPTYMPNAVAGDTGHNPQKVRTSKNVGFSGYQERVHIATAESLIWRRMVIWSYNRLENTAGPTKTDDQGTSYTTRQLTPLQLNEGVRAFLFRGTQGIDYTENTLHEAPLNSDHFTVAYDRTRVLQPRRPTGDEYGHIFNMKFWNPGGRIIYSDDEDGLQKGPLVNGWSSLGRVSKGNMYIFDVFSTGYSLSSNTPSIARFAPTGTRYWTE

SEQ ID NO: 198 - protein, 305 aa, Artificial Sequence
  SOURCE 1..305: /mol_type="protein" /note="subject" /organism="Artificial Sequence"
RSSRFRARRPIKTSRRGGVSKPRRRSYSAKKRTYRKKASMSKRSILNTTSRKKRNGMLTFSNTTNSGASTAPAAAPVYVNAVLGGTFIWCPTAMNLVAQSLISNMSSHTATTCYMRGLSEHIRIQTSSGIPWFHRRVCFTWKGLGPFNVMATESPTSDFPWLPYQDSSNGVQRLFFNENVNNMPQTINRQRNILFKGAENVDWTDPIIAPLDTGRITVKFDKTWTMQSGNTNGIVRERKLWHPMNHNLVYDDDEYGDIESGSWFSTDSKAGMGDYYVMDIIQGGQGGTASDLLRMTANSTMYWHE

SEQ ID NO: 199 - protein, 151 aa, Artificial Sequence
  SOURCE 1..151: /mol_type="protein" /note="query" /organism="Artificial Sequence"
PLCCRLGRERHSDGGIHYHIYLGFDKIVTVNSATAFDYFGAHGNIKSIRRTPHKVFDYVGKDGDIRLEHGEPPADARSCDGDNSNKWADIISCDTKESFLSAVRQQAPRDWLLSNQRIIEYANFYYPDEKPEYEAPPIIVERERYPEISEW

SEQ ID NO: 200 - protein, 150 aa, Artificial Sequence
  SOURCE 1..150: /mol_type="protein" /note="subject" /organism="Artificial Sequence"
PAECIIGRENHADGGIHLHAFVDFGKRVDIRDNRRFDVEGFHPNIAPCGRTPQKMLDYAIKDGDVVAGGLNPILDLPDAETDSIWHRIANAPSVDEFWAITRELAPRALLCNHQSLRAYAEWHYRPVATRYEHPHGLSLRTDHVPQLDEW

SEQ ID NO: 201 - protein, 179 aa, Artificial Sequence
  SOURCE 1..179: /mol_type="protein" /note="query" /organism="Artificial Sequence"
MPRRFQVRARNLIITFPQVPEHLQHEFDAGTPFLERVTANFGNPLCCRLGRERHSDGGIHYHIYLGFDKIVTVNSATAFDYFGAHGNIKSIRRTPHKVFDYVGKDGDIRLEHGEPPADARSCDGDNSNKWADIISCDTKESFLSAVRQQAPRDWLLSNQRIIEYANFYYPDEKPEYEAP

SEQ ID NO: 202 - protein, 184 aa, Artificial Sequence
  SOURCE 1..184: /mol_type="protein" /note="subject" /organism="Artificial Sequence"
MSRQFCLKDAKYCLLTYPQIPETEAYEFPELASELFSSERVDANYVIGRELHADGGYTSHCFLDFGRKFSSRDTRIFDIQGHHPNIERVGRTPRTAYNYTIKDNDVVARSGEYSGPPENNNSRERQSGNDTSSDWATILCAESRDEFFDLCKSLQPRSLACSFLSLTRYADWRYRPVPTPYQHP

SEQ ID NO: 203 - protein, 151 aa, Artificial Sequence; identical to SEQ ID NO: 199
  SOURCE 1..151: /mol_type="protein" /note="query" /organism="Artificial Sequence"

SEQ ID NO: 204 - protein, 153 aa, Artificial Sequence
  SOURCE 1..153: /mol_type="protein" /note="subject" /organism="Artificial Sequence"
PAECIIGREAHADGGTHLHAFCDFGERFYTADPRRFDVDGYHPNVQPFGRTPYKGWDYAIKDGDVVCGGLERPGTGPGTDVSGAGSQWDRIVGAETPDEFWRLIRELAPRTLLTNFNSVRAYADWHYRPVVAPYESPPEIEFDLSGVEELREW

SEQ ID NO: 205 - protein, 86 aa, Artificial Sequence
  SOURCE 1..86: /mol_type="protein" /note="query" /organism="Artificial Sequence"
MDEFSDDCQYAVFDDIQGGFEYFHSYKGWLGAQKQFVITDKYRKKRTIYWGKPSIMCMNEDPHFAKGVDYDWLMNNCHIINVVDPI

SEQ ID NO: 206 - protein, 86 aa, Artificial Sequence
  SOURCE 1..86: /mol_type="protein" /note="subject" /organism="Artificial Sequence"
LDESLEDVDYAVFDDMQGGLEFFHAYKFWLGAQKQFYATDKYRGKQLVNWGRPSIYISNTNPLADKGADVDWLMGNCVIVHVDRPI

SEQ ID NO: 207 - protein, 88 aa, Artificial Sequence
  SOURCE 1..88: /mol_type="protein" /note="query" /organism="Artificial Sequence"
MDEFSDDCQYAVFDDIQGGFEYFHSYKGWLGAQKQFVITDKYRKKRTIYWGKPSIMCMNEDPHFAKGVDYDWLMNNCHIINVVDPICI

SEQ ID NO: 208 - protein, 88 aa, Artificial Sequence
  SOURCE 1..88: /mol_type="protein" /note="subject" /organism="Artificial Sequence"
LEEELEGVDYAIFDDMQGGLKFFHSYKFWLGAQSQFWATDKYRGKKLIHWGRPSIYICNQNPLCDEGVDHDWLIGNCDFVEITESLLV

SEQ ID NO: 209 - protein, 81 aa, Artificial Sequence
  SOURCE 1..81: /mol_type="protein" /note="query" /organism="Artificial Sequence"
DDCQYAVFDDIQGGFEYFHSYKGWLGAQKQFVITDKYRKKRTIYWGKPSIMCMNEDPHFAKGVDYDWLMNNCHIINVVDPI

SEQ ID NO: 210 - protein, 81 aa, Artificial Sequence
  SOURCE 1..81: /mol_type="protein" /note="subject" /organism="Artificial Sequence"
DDAQYAVLDDIQGNFQFFPAYKGWLGAQESFTVTDKYRGKTTITWGRPTIWLMNEDPEEVGHVDLNWLRGNCTIVHLTQSL

SEQ ID NO: 211 - DNA, 2259 bp, Artificial Sequence
  source 1..2259: /mol_type="DNA" /note="MSSI2.225" /organism="Artificial Sequence"
ttcctaatcagctgttcgatcagaccaccgaaggtggatgtcgacgcgtcatcggcccacttctcggggtcactaatgcccgagatgagctgcaatcttacgtcttccggggtcaggaagattctgattgggcagatcagtttactgccccccttgatactcgtcgcattacggttaagtccgacaaactccgcgtcatccgccccggtaatgaaacaggtgcttcgcgcttgtttaagttttggtaccccattcgtcgtaccatctcttacgaagatgaccttgagtccgacgttgtcggtgatcggcccttttctaccgcaggtttacgaggtgttggggatatgtacgtcatggatataatgggtattacgaatttggtgaatgatgcacctccaacgtcctacaggttcggtcctgagggcagcttttattggcatgagcggtaaattaggagactatggggctatctaggtacacgaaatcgcagttggcattaagccactcggtgtcaacaccaagctcgtcacgtgggtcggagttagatagccaaattgagggccgagcccagtgtaccaactttttccccttgtacttatccgtgacgtagaactgcttttgatgacctaaccagaatttgtagctgggaaggaatttaattcctccgaagtcgtcaaagatggcgtactcaaccccatcaaggttttcgtccaagctaaagaggcctccgaagtaagcatggtttcccaggcttctagcccaaatggtttttcccattctggaaggcccgtataccacaagtgattttcttcgttctgtatatcgaagtcagcatccagatttgttgatgcgcactcgagcgaggcgctgcgcgaggcccccgccgagcatggaggcgcgcgtagccgccgactgcagccgctgcgacgtgcatgataacttacctccagtttcacctcgtccaagattttgttgtacccattgattgagttcagccacccaagacgtatcgatgttaactccctccggtgtctcatacgggactctgattggtgggaatttccaggctgcgtatgccctgagctgggtgaaggaggtgaccaatgagcgtggagccaggcgtttgcataggtcccaaaactcttgctcactctcagcattgatgatttcagcccacaccccactagttgcatccactctgcctgcaacaggtcgctcgagtcccccagcaacaacatctccatctttgattgcataatcaaacccctcttctggtgttccgcgagaaggcgatacatttgggtggcatccttcaacatcgaatgcacgcgcgttccgggtcctatatttgactccgaagtcgacaaaagcgtgcagatgaagacccccatctgcgtgattctctcggccgatgatgcattcagctccaagtcccgcaagatgattgaccactgcaaaagggtcgaggtctccacattgtggataggtgagcaaggcgtaccgtgcttgaaatcgaaaagaggacatagttcgttgttgcacattttccttgggtccaagtctgggcagttaatgttatatgcccagacggacccagacccgggtccttcgaactataaatacccctcgctcgtccccaacctcctcgtttttttgtatgcgcgatttatcatgtctgccttgatccaccccgttgcctgcaatcggacttgccaagactacgtcaaccacgctagacacgaatgttgtttagtgtgtaaccctccgccacccccttcatctcctactgtcgcacattgttcagaatgtcggtcgcccgtcgatctggtcgaagaactcgcaaagctttccgccgcggtggtagagctacaagatctcgtggccgaagtacacgccgctcttctaggcgaagagtcagacggcgaactatgactacccgacgtgtcctcaacataaccactcgtaagaaggtggataacatgttgcctgttgttgttgccgaggataacacgactactgtggggccttacacgtccgtgtcacccctcctttcccttttcgttcccaatgcccgcacgacccgaacccctgttaccaatcctgccgtccgaaattcctcggatattttcgcggtcggatatagggagcgcgtccgcattgatcttatgggtggtggaacttttatgtggcgccgcatcgtcttcatgttgaagggatccgatttgagagttgctatgaattccagtgattcaggcaaca

SEQ ID NO: 212 - DNA, 335 bp, Artificial Sequence
  source 1..335: /mol_type="DNA" /note="query" /organism="Artificial Sequence"
ccactctgcctgcaacaggtcgctcgagtcccccagcaacaacatctccatctttgattgcataatcaaacccctcttctggtgttccgcgagaaggcgatacatttgggtggcatccttcaacatcgaatgcacgcgcgttccgggtcctatatttgactccgaagtcgacaaaagcgtgcagatgaagacccccatctgcgtgattctctcggccgatgatgcattcagctccaagtcccgcaagatgattgaccactgcaaaagggtcgaggtctccacattgtggataggtgagcaaggcgtaccgtgcttgaaatcgaaaagaggacata

SEQ ID NO: 213 - DNA, 338 bp, Artificial Sequence
  source 1..338: /mol_type="DNA" /note="subject" /organism="Artificial Sequence"
ccactccgccatcatcagcgggtctgtccagtcctccagcaacaacatccccatctttgattgcatagtcgtatccgccagctgggcgtccccgagatggttcaacattcgggtggtgtccttgcacatcgaagacgcgtacgttccgcgtactaaatttgactccgaagtcgacgaaagcatggagatgaattccttcatcagcgtgagtctctcgtccaatgatgcactctgctctaaggcctgataggtggtcagacacagcaaacgggtcgaggtctccacactgggcgtaagtgagtaaggcatatctggcctggaatctgaatgatgacata

SEQ ID NO: 214 - DNA, 307 bp, Artificial Sequence
  source 1..307: /mol_type="DNA" /note="query" /organism="Artificial Sequence"
acaccaagctcgtcacgtgggtcggagttagatagccaaattgagggccgagcccagtgtaccaactttttccccttgtacttatccgtgacgtagaactgcttttgatgacctaaccagaatttgtagctgggaaggaatttaattcctccgaagtcgtcaaagatggcgtactcaaccccatcaaggttttcgtccaagctaaagaggcctccgaagtaagcatggtttcccaggcttctagcccaaatggtttttcccattctggaaggcccgtataccacaagtgattttcttcgttctgtat

SEQ ID NO: 215 - DNA, 307 bp, Artificial Sequence
  source 1..307: /mol_type="DNA" /note="subject" /organism="Artificial Sequence"
accccatgctcctcgcgtgggtcctcattgttgatccatattgatggtctgccccattcaaccaactttttccccttgtacttgtctgtgacgtaaaactgcttctggtgtcccatccaaaatttgtaagatgggaggaattttaaacctccaaaatcatcaaacaccgcatatgtggccgagcttatgtcctcgtccattgagaaaagccctccgaaataggcatggtctcctagtgacctggcccacacagtcttacccgttcgggttggaccatatagcactagtgatttccctcttactatat

SEQ ID NO: 216 - DNA, 277 bp, Artificial Sequence
  source 1..277: /mol_type="DNA" /note="query" /organism="Artificial Sequence"
tcgagtcccccagcaacaacatctccatctttgattgcataatcaaacccctcttctggtgttccgcgagaaggcgatacatttgggtggcatccttcaacatcgaatgcacgcgcgttccgggtcctatatttgactccgaagtcgacaaaagcgtgcagatgaagacccccatctgcgtgattctctcggccgatgatgcattcagctccaagtcccgcaagatgattgaccactgcaaaagggtcgaggtctccacattgtggataggtgagca

SEQ ID NO: 217 - DNA, 277 bp, Artificial Sequence
  source 1..277: /mol_type="DNA" /note="subject" /organism="Artificial Sequence"
tcgagtcctccagcaacaacatctccgtccttgatcgcataagttgcacccttttccggtgttgagtaaccgcgtacgacatttgggtggcgtccgtccacatcgaatacgcggacatttcttgactcaaacttccgttcgaacatgaagaaagcgtgcaggtgaagtcctccatcagcgtgctcttctcggccaatgatgcactcagctcccaggcgtccaagatggtcgttaacttcccaggggtccaggtctccggactgggggaacgtgagca

SEQ ID NO: 218 - DNA, 276 bp, Artificial Sequence
  source 1..276: /mol_type="DNA" /note="query" /organism="Artificial Sequence"
agtcccccagcaacaacatctccatctttgattgcataatcaaacccctcttctggtgttccgcgagaaggcgatacatttgggtggcatccttcaacatcgaatgcacgcgcgttccgggtcctatatttgactccgaagtcgacaaaagcgtgcagatgaagacccccatctgcgtgattctctcggccgatgatgcattcagctccaagtcccgcaagatgattgaccactgcaaaagggtcgaggtctccacattgtggataggtgagcaag

SEQ ID NO: 219 - DNA, 276 bp, Artificial Sequence
  source 1..276: /mol_type="DNA" /note="subject" /organism="Artificial Sequence"
aggcccccacaaatgacatctccatctttgatcgcgtagtcataccccttctccggagtccctcgagactttgtaatgtttgggtggtgaccatcgacatcgaatacatcagcctttctactgcgaaacttccgtccgaactctgcaaagcagtgtaggtgaatgcctccatcctcgtgatgctctcttccaatgatgcactcagctcccagaagtgaaagtttatccataactcggaaagcatcgagctctccacattgtgcgtatgtgagcaag

SEQ ID NO: 220 - protein, 256 aa, Artificial Sequence
  SOURCE 1..256: /mol_type="protein" /note="query" /organism="Artificial Sequence"
RRVLNITTRKKVDNMLPVVVAEDNTTTVGPYTSVSPLLSLFVPNARTTRTPVTNPAVRNSSDIFAVGYRERVRIDLMGGGTFMWRRIVFMLKGSDLRVAMNSSDSGNIPNQLFDQTTEGGCRRVIGPLLGVTNARDELQSYVFRGQEDSDWADQFTAPLDTRRITVKSDKLRVIRPGNETGASRLFKFWYPIRRTISYEDDLESDVVGDRPFSTAGLRGVGDMYVMDIMGITNLVNDAPPTSYRFGPEGSFYWHER

SEQ ID NO: 221 - protein, 265 aa, Artificial Sequence
  SOURCE 1..265: /mol_type="protein" /note="subject" /organism="Artificial Sequence"
  VARIANT 234: / unknown or other unknown or other unknown or other
  VARIANT 93: unknown or other
  VARIANT 122: unknown or other
RRILNVASIKKRDNMLSMVQTSDQAPPTIGPITVGTGFASLYMPSARPLGPANDVGESTRQRRDTFSVGYKERVQVDIHGGGVWKWRRVVFTXKGDQLYNKGEFIGDWTQPFESKAVKPSPXDPNPLGVDMVRLIGQPTTEQHNAIRDLIWDGHEGIDWTSEFTAKVSTTRITVLSDKTYHFNPGNESGMSRTFRLWYPTRKRLIYDDDERGGAVFSRGSPVSVTSRQGMGDLXIYDIAYAVVPSAGNPGSMTWAPEGTYYWHER

SEQ ID NO: 222 - protein, 300 aa, Artificial Sequence
  SOURCE 1..300: /mol_type="protein" /note="query" /organism="Artificial Sequence"
MSVARRSGRRTRKAFRRGGRATRSRGRSTRRSSRRRVRRRTMTTRRVLNITTRKKVDNMLPVVVAEDNTTTVGPYTSVSPLLSLFVPNARTTRTPVTNPAVRNSSDIFAVGYRERVRIDLMGGGTFMWRRIVFMLKGSDLRVAMNSSDSGNIPNQLFDQTTEGGCRRVIGPLLGVTNARDELQSYVFRGQEDSDWADQFTAPLDTRRITVKSDKLRVIRPGNETGASRLFKFWYPIRRTISYEDDLESDVVGDRPFSTAGLRGVGDMYVMDIMGITNLVNDAPPTSYRFGPEGSFYWHER

SEQ ID NO: 223 - protein, 302 aa, Artificial Sequence
  SOURCE 1..302: /mol_type="protein" /note="subject" /organism="Artificial Sequence"
MAYARRRFTSSRARKPIRRSRRPAGKRRSYRRSTRKRGMSTRTLLNKTSQKKRDNMLSFSNTTAEDPFSTDYTIGPAVMRRPVGADLPAEFIYVWNATGRPHELSTGFRGSKIDTSLRTNTTIFAVGLKERIKLETNNSAPWRWRRICFTSKNDYGEADPDESDYFRRTSNGMVRLLRAQSQAEEINDDVFDGQRNVDWLSAITAPINRRHVSVHYDRTRTIQSGNQSGVTRTYRQWHPMRKNVVYADEQAGEGMVDSGVSVTGKVGMGNYYVMDIFTKHGLNDDQSTLSYEPESTFFWHEK

SEQ ID NO: 224 - protein, 261 aa, Artificial Sequence
  SOURCE 1..261: /mol_type="protein" /note="query" /organism="Artificial Sequence"
RTMTTRRVLNITTRKKVDNMLPVVVAEDNTTTVGPYTSVSPLLSLFVPNARTTRTPVTNPAVRNSSDIFAVGYRERVRIDLMGGGTFMWRRIVFMLKGSDLRVAMNSSDSGNIPNQLFDQTTEGGCRRVIGPLLGVTNARDELQSYVFRGQEDSDWADQFTAPLDTRRITVKSDKLRVIRPGNETGASRLFKFWYPIRRTISYEDDLESDVVGDRPFSTAGLRGVGDMYVMDIMGITNLVNDAPPTSYRFGPEGSFYWHER

SEQ ID NO: 225 - protein, 278 aa, Artificial Sequence
  SOURCE 1..278: /mol_type="protein" /note="subject" /organism="Artificial Sequence"
RKMSKRRILNITSTKKKDTMTGYTNSTPANQTGGTVYSTDPAIVTGGLNANQCNAFLWCATARTNQVINPTQNTLVPGNKFYTACRTDSNPYMVGLSEKIEIQCNSGMPWQWRRICWTQKGGQGLPANSTSFNLSQQNAITGWNRVMNQVAGNPGTGDQYNLFHHIFRGQVGSDWVDVMTAPLDPQHITVKYDKVVTLASGNEEGFIRAYRRWHPMKKTLSYADEEYGNVENADAFSQVGKKGMGDYYVLDLFRARQGAQTNDSISIRPCATLYWHEK

SEQ ID NO: 226 - protein, 195 aa, Artificial Sequence
  SOURCE 1..195: /mol_type="protein" /note="query" /organism="Artificial Sequence"
MSSFRFQARYALLTYPQCGDLDPFAVVNHLAGLGAECIIGRENHADGGLHLHAFVDFGVKYRTRNARAFDVEGCHPNVSPSRGTPEEGFDYAIKDGDVVAGGLERPVAGRVDATSGVWAEIINAESEQEFWDLCKRLAPRSLVTSFTQLRAYAAWKFPPIRVPYETPEGVNIDTSWVAELNQWVQQNLGRGETGG

SEQ ID NO: 227 - protein, 198 aa, Artificial Sequence
  SOURCE 1..198: /mol_type="protein" /note="subject" /organism="Artificial Sequence"
MSSFRFQARYALLTYAQCGDLDPFAVSDHLSGLRAECIIGRETHADEGIHLHAFVDFGVKFSTRNVRVFDVQGHHPNVEPSRGRPAGGYDYAIKDGDVVAGGLDRPADDGGVGVSKTTQKWATIVGAQTRDEFWALLAELDPGAMVRSFTQCRAYADHRFRESPERYVTPESIIIDTGHVDGLNEWALSNIVGHRRGG

SEQ ID NO: 228 - protein, 220 aa, Artificial Sequence
  SOURCE 1..220: /mol_type="protein" /note="query" /organism="Artificial Sequence"
SFRFQARYALLTYPQCGDLDPFAVVNHLAGLGAECIIGRENHADGGLHLHAFVDFGVKYRTRNARAFDVEGCHPNVSPSRGTPEEGFDYAIKDGDVVAGGLERPVAGRVDATSGVWAEIINAESEQEFWDLCKRLAPRSLVTSFTQLRAYAAWKFPPIRVPYETPEGVNIDTSWVAELNQWVQQNLGRGETGGKLSCTSQRLQSAATRASMLGGGLAQRL

SEQ ID NO: 229 - protein, 216 aa, Artificial Sequence
  SOURCE 1..216: /mol_type="protein" /note="subject" /organism="Artificial Sequence"
TFRLQSRYVLLTYAQCGDLDPWLVHNHVVAFPAECIIGRENHADGGIHLHAFVDFGKRVDIRDNRRFDVEGFHPNIAPCGRTPQKMLDYAIKDGDVVAGGLNPILDLPDAETDSIWHRIANAPSVDEFWAITRELAPRALLCNHQSLRAYAEWHYRPVATRYEHPHGLSLRTDHVPQLDEWVRDNLSGSSKSYTYTRSASGRASLPSGGPSLVQSL

SEQ ID NO: 230 - protein, 212 aa, Artificial Sequence
  SOURCE 1..212: /mol_type="protein" /note="query" /organism="Artificial Sequence"
FRFQARYALLTYPQCGDLDPFAVVNHLAGLGAECIIGRENHADGGLHLHAFVDFGVKYRTRNARAFDVEGCHPNVSPSRGTPEEGFDYAIKDGDVVAGGLERPVAGRVDATSGVWAEIINAESEQEFWDLCKRLAPRSLVTSFTQLRAYAAWKFPPIRVPYETPEGVNIDTSWVAELNQWVQQNLGRGETGGKLSCTSQRLQSAATRASMLG

SEQ ID NO: 231 - protein, 212 aa, Artificial Sequence
  SOURCE 1..212: /mol_type="protein" /note="subject" /organism="Artificial Sequence"
FRFAAKYGLLTYPQCGDLDPWAVNDMLGRLGAECVIGRENHQAGGVHLHAFFMFERKFESRNVRVFDVDGHHPNIVRGYSTPEDGWAYATKDGDVVAGALECPRPRTEVSESSSKWARAILAETREEFFAIVAELDPRALCVSFGSLRAYADWKYRPARDPYITPEGISFDTSELPELDLWVQQTLSGLSTGKQPPPSAPLRGVPEQISARG

SEQ ID NO: 232 - protein, 107 aa, Artificial Sequence
  SOURCE 1..107: /mol_type="protein" /note="query" /organism="Artificial Sequence"
MGKTIWARSLGNHAYFGGLFSLDENLDGVEYAIFDDFGGIKFLPSYKFWLGHQKQFYVTDKYKGKKLVHWARPSIWLSNSDPRDELGVDTEWLNANCDFVYLDSPIV

SEQ ID NO: 233 - protein, 110 aa, Artificial Sequence
  SOURCE 1..110: /mol_type="protein" /note="subject" /organism="Artificial Sequence"
TGKTVWARSLGDHAYFGGLFSMDEDISSATYAVFDDFGGLKFLPSYKFWMGHQKQFYVTDKYKGKKLVEWGRPSIWINNEDPREEHGVRCDEIEWLEQNCIFIRLDSTIV

SEQ ID NO: 234 - protein, 107 aa, Artificial Sequence; identical to SEQ ID NO: 232
  SOURCE 1..107: /mol_type="protein" /note="query" /organism="Artificial Sequence"

SEQ ID NO: 235 - protein, 108 aa, Artificial Sequence
  SOURCE 1..108: /mol_type="protein" /note="subject" /organism="Artificial Sequence"
LGKTLWARSLGNHAYFGGLFSLEEELEGVDYAIFDDMQGGLKFFHSYKFWLGAQSQFWATDKYRGKKLIHWGRPSIYICNQNPLCDEGVDHDWLIGNCDFVEITESLL

SEQ ID NO: 236 - protein, 106 aa, Artificial Sequence
  SOURCE 1..106: /mol_type="protein" /note="query" /organism="Artificial Sequence"
MGKTIWARSLGNHAYFGGLFSLDENLDGVEYAIFDDFGGIKFLPSYKFWLGHQKQFYVTDKYKGKKLVHWARPSIWLSNSDPRDELGVDTEWLNANCDFVYLDSPI

SEQ ID NO: 237 - protein, 107 aa, Artificial Sequence
  SOURCE 1..107: /mol_type="protein" /note="subject" /organism="Artificial Sequence"
LGKTLWARSLGRHAYFGGLFCLDESLEDVDYAVFDDMQGGLEFFHAYKFWLGAQKQFYATDKYRGKQLVNWGRPSIYISNTNPLADKGADVDWLMGNCVIVHVDRPI

SEQ ID NO: 238 - protein, 87 aa, Artificial Sequence
  SOURCE 1..87: /mol_type="protein" /note="query" /organism="Artificial Sequence"
TSSGVRKILIGQISLLPPLILVALRLSPTNSASSAPVMKQVLRACLSFGTPFVVPSLTKMTLSPTLSVIGPFLPQVYEVLGICTSWI

SEQ ID NO: 239 - protein, 91 aa, Artificial Sequence
  SOURCE 1..91: /mol_type="protein" /note="subject" /organism="Artificial Sequence"
TSSGVKIVLTIDSSLLDHLFLALPRSSPHQEALAIFLLVPECCVALGACRIPSLALRFAEAVTGLSKGSSNILGPFLEQIVQMLKTCVSAI

SEQ ID NO: 240 - DNA, 1626 bp, Artificial Sequence
  source 1..1626: /mol_type="DNA" /note="MSSI1.162" /organism="Artificial Sequence"
gacttctgattgattgatgcctgccgacttttgataattttttgatagatgatttttcttgactgaaataaaaaaaccccttattgttgtaagtgcttggttcacaacttaataagaggttttaattatgatgtcacatgatggcacacctgtcaattttttgtccgatattcaacccagtgagaaaagctgggacactcaccgagccgaagccgaaagcgtccgattgctttacagtctttcgactgagttcaccaaatacgctagccgtatttatgactgttcccaaatcctaaaatttgcccctacccctgataagctggtacttaaacacgcctttttctgtcgtgttaggtattgccctgtttgccagtggcgtaggtcgttattatggcgggcggtcatgtttcagcagttaccagcaatcaaagagaagtaccctagttatcgttgggtgtttcttacccttactgtcaaaaatcccccagttactgaattaagggacaccttaaaggctatgaattcagcttggcaacgcctagcacaaactaaacgctttaaaggggtcgttaaaggctttattcgcacaaccgaagttacaaggggtaaagatggcgacatgatggctcacccccatttccatgcgctgttattagttcaaagtaattatttcactacaaattatattaaacaaaatgattgggtcgaaatgtggcaaaaggcgttaagggtcgattatgccccatcggtcaacgtaaaagccgttaaaccccctaaaaagggtgaaaaggataatctcgataaggcgatatgtgaaacgctcaaatatagcgttaaaccgtctgatattgccaaagatgacgatgggggcgaatggttgcatgaaatgaccagacaaaccctaaatatgcgttttattgccactggtggcattttgaagggtgtacttaaacccgatgagcaagtaacacaacaagaaatgcttacccccactggtgaagatgaagcaccaaccgaacaaaaacggattggatttagattttacccccatcatgggcgttatgttttttcgccagctatacgaatttttgacttgctgtttttgcaagtcgtaagttcgcccttatagcaaatgtgttgtgcctgtaagtgctgtaaggcatatccagcgttagcaataaacggctttatcgtttattgcgttagcgtctttatatccccaacctttccccctttgaagtcccagcttttttttgtggctgttctattgttgctctttattgaccttacgccacataaaaaaagtgggttacatatcggttgaatttgggttgcaatagtctagggacattcaaaaataatccttcttggtagtattacgaaatctcatgtaatccgcattggtggcggtttacccaaaaacaaaaacaagaaaaattcgtcttgcgaatttttattgctttttgctttttggggtataaaaacctatagaaaaactataaaaaacctatagaattataggtgcttactgggggtttgccttgtatttattattaagggataactctgattttattttatatgattttttatactggcaaacctgttgaataccgcttaaatact

SEQ ID NO: 241 - DNA, 273 bp, Artificial Sequence
  source 1..273: /mol_type="DNA" /note="query" /organism="Artificial Sequence"
aaacacgcctttttctgtcgtgttaggtattgccctgtttgccagtggcgtaggtcgttattatggcgggcggtcatgtttcagcagttaccagcaatcaaagagaagtaccctagttatcgttgggtgtttcttacccttactgtcaaaaatcccccagttactgaattaagggacaccttaaaggctatgaattcagcttggcaacgcctagcacaaactaaacgctttaaaggggtcgttaaaggctttattcgcacaaccgaagttaca

SEQ ID NO: 242 - DNA, 273 bp, Artificial Sequence
  source 1..273: /mol_type="DNA" /note="subject" /organism="Artificial Sequence"
aaacaagcctttttttgccgtgttcgttactgcggtatgtgccaatggcgtaggtcattactctggaaagccttgatgtataaaacatacgatgaaattatgcagacacacccgacacatcgctttgtgtttttaaccctgacgcttaaaaatccgcctatcggtgacttgcgcgaaaccttgcagcacatgaataaatcatggcaacgcttaaaagatcgtaaagaatttatagcaggcgttgaaggttgggtacgcacaacggaagtcaca

SEQ ID NO: 243 - DNA, 89 bp, Artificial Sequence
  source 1..89: /mol_type="DNA" /note="query" /organism="Artificial Sequence"
aattatattaaacaaaatgattgggtcgaaatgtggcaaaaggcgttaagggtcgattatgccccatcggtcaacgtaaaagccgttaa

SEQ ID NO: 244 - DNA, 89 bp, Artificial Sequence
  source 1..89: /mol_type="DNA" /note="subject" /organism="Artificial Sequence"
aattatattaatcaagaagaatggacgagactgtggcgaaaggcgttaaaagtcgattatgagccagtggtgcatgtgcaagtcgttaa

SEQ ID NO: 245 - protein, 313 aa, Artificial Sequence
  SOURCE 1..313: /mol_type="protein" /note="query" /organism="Artificial Sequence"
VNFLSDIQPSEKSWDTHRAEAESVRLLYSLSTEFTKYASRIYDCSQILKFAPTPDKLVLKHAFFCRVRYCPVCQWRRSLLWRAVMFQQLPAIKEKYPSYRWVFLTLTVKNPPVTELRDTLKAMNSAWQRLAQTKRFKGVVKGFIRTTEVTRGKDGDMMAHPHFHALLLVQSNYFTTNYIKQNDWVEMWQKALRVDYAPSVNVKAVKPPKKGEKDNLDKAICETLKYSVKPSDIAKDDDGGEWLHEMTRQTLNMRFIATGGILKGVLKPDEQVTQQEMLTPTGEDEAPTEQKRIGFRFYPHHGRYVFSPAHTNF

SEQ ID NO: 246 - protein, 299 aa, Artificial Sequence
  SOURCE 1..299: /mol_type="protein" /note="subject" /organism="Artificial Sequence"
INFLTEISPHEVSWDEHRSDAESVKILYNYSVELAKYADRINGCSGILKFGVSPNQGKLVLKQAFFCRVRHCPVCQWRRSLLWRAVMFQQLPKIQKLYPTHRWVFLTMTVRNPPIIELRDTLKHMNESWQRLIQTKAFKSGVAGFIRTTEVTRGKDAEMMSHPHYHALLLVKPGYFSKYYINQSEWVEMWAKALRADYLPSVNVKAIRAGNNEKSKKALEKQICETLKYSVKPSDLAVERDKGAWLHEMTKQVHKMRFVATGGVLKGILKPDDEITNEEMISSSEETEDVGEGRVAFQF

SEQ ID NO: 247 - protein, 313 aa, Artificial Sequence; identical to SEQ ID NO: 245
  SOURCE 1..313: /mol_type="protein" /note="query" /organism="Artificial Sequence"

SEQ ID NO: 248 - protein, 315 aa, Artificial Sequence
  SOURCE 1..315: /mol_type="protein" /note="subject" /organism="Artificial Sequence"
INFLTEISPHEVSWDEHRSDAESVKILYNYSVELAKYADRINGCSGILKFGVSPNQGKLVLKQAFFCRVRHCPVCQWRRSLLWRAVMFQQLPKIQKLYPTHRWVFLTMTVRNPPIIELRDTLKHMNESWQRLIQTKAFKSGVAGFIRTTEVTRGKDAEMMSHPHYHALLLVKPGYFSKYYINQSEWVEMWAKALRADYLPSVNVKAIRAGNNEKSKKALEKQICETLKYSVKPSDLAVERDKGAWLHEMTKQVHKMRFVATGGVLKGILKPDDEITNEEMISSSEETEDVGEGRVAFQFNSEYRRYVYAPKFNEY